European Patent Specification EP 3 765 101 B1, published October 15, 2025. Title: Methods and Compositions. Applicant: Imperial Innovations Limited. The sequence listing filed with the application follows.

SEQUENCE LISTING (173 sequences)

SEQ ID NO: 1 - protein, 135 aa, Artificial Sequence
  SynRFR24.new_caps solenoid domain UNITSn
ASLTGADLSYANLHHANLSRANLRSADLRNANLSHANLSGANLEEANLEAANLRGADLHEANLSGADLQEANLTQANLKDANLSDANLEQADLAGADLQGAVLDGANLHGANLNNANLSEAMLTRANLEQADLSG

SEQ ID NO: 2 - protein, 30 aa, Artificial Sequence
  Cap sequence 1 SynRFR24.new_caps
RMRRDEILEEYRRGRRNFQHINLQEIELTN

SEQ ID NO: 3 - protein, 46 aa, Artificial Sequence
  Cap sequence 2 SynRFR24.new_caps
ARTTGARLDDADLRGATVDPVLWRTASLRGAKMEEEQRREYERARG

SEQ ID NO: 4 - protein, 30 aa, Artificial Sequence
  Cap sequence 1 original SynRFR24.1
HMNVGEILRHYAAGKRNFQHINLQEIELTN

SEQ ID NO: 5 - protein, 52 aa, Artificial Sequence
  Cap sequence 2 original SynRFR24.1
ARTTGARLDDADLRGATVDPVLWRTASLVGARVDVDQAVAFAAAHGLCLAGG

SEQ ID NO: 6 - protein, 235 aa, Artificial Sequence
  SynRFR24.new_caps solenoid domain plus both caps plus his tag
MGSSHHHHHHSSGLVPRGSRMRRDEILEEYRRGRRNFQHINLQEIELTNASLTGADLSYANLHHANLSRANLRSADLRNANLSHANLSGANLEEANLEAANLRGADLHEANLSGADLQEANLTQANLKDANLSDANLEQADLAGADLQGAVLDGANLHGANLNNANLSEAMLTRANLEQADLSGARTTGARLDDADLRGATVDPVLWRTASLRGAKMEEEQRREYERARGKSDDG

SEQ ID NO: 7 - protein, 239 aa, Artificial Sequence
  SynRFR24.1 solenoid domain plus both caps plus his tag
MGSSHHHHHHSSGLVPRGSHMNVGEILRHYAAGKRNFQHINLQEIELTNASLTGADLSYANLHHANLSRANLRSADLRNANLSHANLSGANLEEANLEAANLRGADLHEANLSGADLQEANLTQANLKDANLSDANLEQADLAGADLQGAVLDGANLHGANLNNANLSEAMLTRANLEQADLSGARTTGARLDDADLRGATVDPVLWRTASLVGARVDVDQAVAFAAAHGLCLAGGSGC

SEQ ID NO: 8 - protein, 135 aa, Artificial Sequence
  rfr_ref_minprep_ren_neg_num_20_0004 UNITSn
AKLAKANLSNANLKKARLQNANLANAKLQNANLENANLAGANLKKANLRGANLHGADLAGANLKGADLREADLRNADLRKANLTGAKLKNAKLEGANLADATLKDANLHGAKLKNANLARANLERADLRNADLTG

SEQ ID NO: 9 - protein, 135 aa, Artificial Sequence
  rfr_ref_minprep_ren_neg_num_21_0003 UNITSn
AKLAGADLSNAKLHNANLENADLKGANLAGANLQKANLHGADLTNADLRKANLANANLANANLEGARLADADLRNADLRGAKLKRADLENADLTGANLKGANLEGARLERANLKKARLQNAKLAGADLRNARLAG

SEQ ID NO: 10 - protein, 135 aa, Artificial Sequence
  rfr_ref_minprep_ren_neg_num_22_0001 UNITSn
ATLAGANLTGAKLHNARLENADLKDAKLARANLQKANLRGANLRNADLREADLANANLARADLTGAKLADADLRNADLREANLKNANLARANLKGANLHGANLHGARLEKANLENANLQNANLQNANLANADLRG

SEQ ID NO: 11 - protein, 135 aa, Artificial Sequence
  rfr_ref_minprep_ren_neg_num_23_0004 UNITSn
AKLAGADLSNADLRNANLQNANLANANLENADLENADLKGARLENANLRRANLRGANLAEARLEKADLRNANLANADLRRANLRNAELQNADLQGANLEGADLTGANLKGAKLKNANLQNARLAKADLRNADLTG

SEQ ID NO: 12 - protein, 135 aa, Artificial Sequence
  rfr_ref_minprep_ren_neg_num_24_0002 UNITSn
AELAGANLAGANLKNANLRNANLKDADLRKANLQKADLKGANLQNARLQGANLENANLAGARLQGANLAKADLRGADLRNANLTNARLEKADLTDADLHGARLQGADLHGANLERARLQNANLAEADLRNANLTG

SEQ ID NO: 13 - protein, 135 aa, Artificial Sequence
  rfr_ref_minprep_ren_neg_num_25_0003 UNITSn
ATLAGADLSNANLKQADLARANLKDANLQNANLKNAKLEGANLAKANLEKANLHGANLARADLTGANLANAKLENADLRKADLTNADLTNADLRGADLEGANLHGANLKGANLRKAKLKRAELQNADLRNADLTG

SEQ ID NO: 14 - protein, 135 aa, Artificial Sequence
  rfr_ref_minprep_ren_neg_num_26_0004 UNITSn
ATLAGAKLRNANLHNARLQNANLANADLQQADLEEANLHGANLANANLEEANLRRADLANADLTGANLANADLRQADLRGANLRNARLQKANLADADLHGADLHGANLEGANLRRARLENAKLANADLRNADLKG

SEQ ID NO: 15 - protein, 135 aa, Artificial Sequence
  rfr_ref_minprep_ren_neg_num_27_0004 UNITSn
ATLAGADLSKANLHRADLKNANLKGANLEKADLREADLHGADLTNANLHGARLARADLANANLKGADLANADLREANLHGADLTNARLQNARLQDADLHGANLTGARLHGADLTNARLQRADLSKADLRNANLEG

SEQ ID NO: 16 - protein, 135 aa, Artificial Sequence
  rfr_ref_minprep_ren_neg_num_28_0002 UNITSn
ATLAGADLRNANLKNANLQKANLANANLRNANLQGADLAKARLENADLHGARLAKANLAGANLHGADLANADLRNANLRNADLRNARLERADLAGADLEGANLHGANLREARLENANLKRANLQNANLANADLTG

SEQ ID NO: 17 - protein, 135 aa, Artificial Sequence
  rfr_ref_minprep_ren_neg_num_29_0005 UNITSn
ATLAGAKLEGADLTRAKLKDANLAKANLRNANLQEANLKGANLRNADLAGANLERANLAKADLHGANLANADLREADLRNANLDNADLRNADLTGADLEGASLHGANLKKARLENARLRRARLENANLAKANLTG

SEQ ID NO: 18 - protein, 135 aa, Artificial Sequence
  rfr_ref_minprep_ren_neg_num_30_0005 UNITSn
ATLAGADLSGADLHNADLQNAKLKGANLEKARLRRANLRGADLTNANLRGADLEEADLAGARLHGANLARARLANADLRNADLRNANLREADLTGANLHGANLHGADLERANLTNADLENARLERANLAEANLQD

SEQ ID NO: 19 - protein, 135 aa, Artificial Sequence
  rfr_ref_minprep_ren_neg_num_31_0005 UNITSn
ATLKGANLQDANLQEANLQNANLQGARLSNADLRRADLEGANLENADLSGARLQEANLAGARLEGADLADADLRGADLRNADLTNARLERANLADADLHGADLHGAKLHGANLERARLENARLENADLRNAKLAG

SEQ ID NO: 20 - protein, 135 aa, Artificial Sequence
  >rfr_ref_minprep_ren_neg_num_32_0001 UNITSn
ATLAGADLSNANLENADLQNADLANAKLQNANLARANLHGADLRNADLEGADLAEANLANANLEGADLANADLRNADLRGANLTNARLQNANLTGANLRGANLHGADLHGAKLRKADLEKARLENADLRKADLKG

SEQ ID NO: 21 - protein, 135 aa, Artificial Sequence
  rfr_ref_minprep_ren_neg_num_33_0004 UNITSn
AKLAGADLRDADLQRANLENADLANAKLKNANLEQANLEGANLENANLAKADLRNANLARADLTGADLSNADLRGADLRKANLTNADLTNADLEGADLTDARLQGANLHGANLTNANLARANLAGADLRNAKLSG

SEQ ID NO: 22 - protein, 135 aa, Artificial Sequence
  rfr_ref_minprep_ren_neg_num_34_0001 UNITSn
ATLSGAKLEGANLKRADLRNANLSKADLRNANLQQANLQGADLENADLQGANLEEANLAKANLTGANLSNADLRKADLRNANLKDADLENADLEGANLHGADLHGAKLHGADLTRADLENARLENADLRNARLNG

SEQ ID NO: 23 - protein, 135 aa, Artificial Sequence
  rfr_ref_minprep_ren_neg_num_35_0005 UNITSn
AELAGADLANANLHRANLENANLANAKLEEANLEEANLAGADLRNANLQRANLARADLAGADLTGANLAEADLREARLQKANLENADLTNADLTGADLEGARLHGANLEGANLTNANLRKANLENADLRNADLTG

SEQ ID NO: 24 - protein, 135 aa, Artificial Sequence
  rfr_ref_minprep_ren_neg_num_36_0005 UNITSn
AELAGADLSGADLTRADLRDANLANADLQEANLAEAKLQGANLENANLARADLSRANLAGADLHGANLAEADLRNADLRNANLQNADLRKARLQGADLEGANLEGANLHGADLENADLARADLQKADLRNANLTG

SEQ ID NO: 25 - protein, 135 aa, Artificial Sequence
  rfr_ref_minprep_ren_neg_num_37_0002 UNITSn
ATLADADLSDARLHRADLQDADLENANLENADLSEANLRGADLRNANLRKADLARADLAGANLHGADLANAKLAEADLRDADLRNANLENADLTGANLQGARLEGAKLHGANLTNANLKDADLSGADLRDANLTG

SEQ ID NO: 26 - protein, 135 aa, Artificial Sequence
  rfr_ref_minprep_ren_neg_num_38_0005 UNITSn
ATLKGANLQGARLHNADLEEAELKDANLAEADLQNANLRRADLTNADLANANLHGANLAEANLHGANLAGADLRNADLENADLRNANLEDADLKGANLHGANLQGANLEGARLQNANLKNARLAEADLRNADLKG

SEQ ID NO: 27 - protein, 135 aa, Artificial Sequence
  rfr_ref_minprep_ren_neg_num_39_0003 UNITSn
AELAGADLSNADLRNAKLENANLADANLENADLENANLRGADLENADLRRADLHGADLAKANLEGANLAEADLRNADLRNANLTNADLKNADLEGADLHGARLEGANLEGANLENADLANADLSDADLRKADLTG

SEQ ID NO: 28 - protein, 135 aa, Artificial Sequence
  rfr_ref_minprep_ren_neg_num_40_0004 UNITSn
AELAGADLSDANLEQANLQNANLANANLENANLQDADLHGARLQNADLRGANLEDADLANARLEGANLAEADLRRADLRGADLTNADLEDADLEGANLHGARLEGANLRGANLTDARLENADLSGADLRNANLEG

SEQ ID NO: 29 - protein, 861 aa, Artificial Sequence
  SynRFR24.new_caps.x4.1 concatemer of four beta solenoid domains, not including N-terminal His tag
RMRRDEILEEYRRGRRNFQHINLQEIELTNASLTGADLSYANLHHANLSRANLRSADLRNANLSHANLSGANLEEANLEAANLRGADLHEANLSGADLQEANLTQANLKDANLSDANLEQADLAGADLQGAVLDGANLHGANLNNANLSEAMLTRANLEQADLSGARTTGARLDDADLRGATVDPVLWRTASLRGAKMEEEQRREYERARGGGGSRMRRDEILEEYRRGRRNFQHINLQEIELTNASLTGADLSYANLHHANLSRANLRSADLRNANLSHANLSGANLEEANLEAANLRGADLHEANLSGADLQEANLTQANLKDANLSDANLEQADLAGADLQGAVLDGANLHGANLNNANLSEAMLTRANLEQADLSGARTTGARLDDADLRGATVDPVLWRTASLRGAKMEEEQRREYERARGGGGSRMRRDEILEEYRRGRRNFQHINLQEIELTNASLTGADLSYANLHHANLSRANLRSADLRNANLSHANLSGANLEEANLEAANLRGADLHEANLSGADLQEANLTQANLKDANLSDANLEQADLAGADLQGAVLDGANLHGANLNNANLSEAMLTRANLEQADLSGARTTGARLDDADLRGATVDPVLWRTASLRGAKMEEEQRREYERARGGGGSRMRRDEILEEYRRGRRNFQHINLQEIELTNASLTGADLSYANLHHANLSRANLRSADLRNANLSHANLSGANLEEANLEAANLRGADLHEANLSGADLQEANLTQANLKDANLSDANLEQADLAGADLQGAVLDGANLHGANLNNANLSEAMLTRANLEQADLSGARTTGARLDDADLRGATVDPVLWRTASLRGAKMEEEQRREYERARGKSDDG

SEQ ID NO: 30 - protein, 880 aa, Artificial Sequence
  SynRFR24.new_caps.x4.1 concatemer of four beta solenoid domains, including N-terminal His ta
MGSSHHHHHHSSGLVPRGSRMRRDEILEEYRRGRRNFQHINLQEIELTNASLTGADLSYANLHHANLSRANLRSADLRNANLSHANLSGANLEEANLEAANLRGADLHEANLSGADLQEANLTQANLKDANLSDANLEQADLAGADLQGAVLDGANLHGANLNNANLSEAMLTRANLEQADLSGARTTGARLDDADLRGATVDPVLWRTASLRGAKMEEEQRREYERARGGGGSRMRRDEILEEYRRGRRNFQHINLQEIELTNASLTGADLSYANLHHANLSRANLRSADLRNANLSHANLSGANLEEANLEAANLRGADLHEANLSGADLQEANLTQANLKDANLSDANLEQADLAGADLQGAVLDGANLHGANLNNANLSEAMLTRANLEQADLSGARTTGARLDDADLRGATVDPVLWRTASLRGAKMEEEQRREYERARGGGGSRMRRDEILEEYRRGRRNFQHINLQEIELTNASLTGADLSYANLHHANLSRANLRSADLRNANLSHANLSGANLEEANLEAANLRGADLHEANLSGADLQEANLTQANLKDANLSDANLEQADLAGADLQGAVLDGANLHGANLNNANLSEAMLTRANLEQADLSGARTTGARLDDADLRGATVDPVLWRTASLRGAKMEEEQRREYERARGGGGSRMRRDEILEEYRRGRRNFQHINLQEIELTNASLTGADLSYANLHHANLSRANLRSADLRNANLSHANLSGANLEEANLEAANLRGADLHEANLSGADLQEANLTQANLKDANLSDANLEQADLAGADLQGAVLDGANLHGANLNNANLSEAMLTRANLEQADLSGARTTGARLDDADLRGATVDPVLWRTASLRGAKMEEEQRREYERARGKSDDG

SEQ ID NO: 31 - protein, 1721 aa, Artificial Sequence
  SynRFR24.new_caps.x8.1 concatemer of eight beta solenoid domains, not including N-terminal His tag
RMRRDEILEEYRRGRRNFQHINLQEIELTNASLTGADLSYANLHHANLSRANLRSADLRNANLSHANLSGANLEEANLEAANLRGADLHEANLSGADLQEANLTQANLKDANLSDANLEQADLAGADLQGAVLDGANLHGANLNNANLSEAMLTRANLEQADLSGARTTGARLDDADLRGATVDPVLWRTASLRGAKMEEEQRREYERARGGGGSRMRRDEILEEYRRGRRNFQHINLQEIELTNASLTGADLSYANLHHANLSRANLRSADLRNANLSHANLSGANLEEANLEAANLRGADLHEANLSGADLQEANLTQANLKDANLSDANLEQADLAGADLQGAVLDGANLHGANLNNANLSEAMLTRANLEQADLSGARTTGARLDDADLRGATVDPVLWRTASLRGAKMEEEQRREYERARGGGGSRMRRDEILEEYRRGRRNFQHINLQEIELTNASLTGADLSYANLHHANLSRANLRSADLRNANLSHANLSGANLEEANLEAANLRGADLHEANLSGADLQEANLTQANLKDANLSDANLEQADLAGADLQGAVLDGANLHGANLNNANLSEAMLTRANLEQADLSGARTTGARLDDADLRGATVDPVLWRTASLRGAKMEEEQRREYERARGGGGSRMRRDEILEEYRRGRRNFQHINLQEIELTNASLTGADLSYANLHHANLSRANLRSADLRNANLSHANLSGANLEEANLEAANLRGADLHEANLSGADLQEANLTQANLKDANLSDANLEQADLAGADLQGAVLDGANLHGANLNNANLSEAMLTRANLEQADLSGARTTGARLDDADLRGATVDPVLWRTASLRGAKMEEEQRREYERARGGGGSRMRRDEILEEYRRGRRNFQHINLQEIELTNASLTGADLSYANLHHANLSRANLRSADLRNANLSHANLSGANLEEANLEAANLRGADLHEANLSGADLQEANLTQANLKDANLSDANLEQADLAGADLQGAVLDGANLHGANLNNANLSEAMLTRANLEQADLSGARTTGARLDDADLRGATVDPVLWRTASLRGAKMEEEQRREYERARGGGGSRMRRDEILEEYRRGRRNFQHINLQEIELTNASLTGADLSYANLHHANLSRANLRSADLRNANLSHANLSGANLEEANLEAANLRGADLHEANLSGADLQEANLTQANLKDANLSDANLEQADLAGADLQGAVLDGANLHGANLNNANLSEAMLTRANLEQADLSGARTTGARLDDADLRGATVDPVLWRTASLRGAKMEEEQRREYERARGGGGSRMRRDEILEEYRRGRRNFQHINLQEIELTNASLTGADLSYANLHHANLSRANLRSADLRNANLSHANLSGANLEEANLEAANLRGADLHEANLSGADLQEANLTQANLKDANLSDANLEQADLAGADLQGAVLDGANLHGANLNNANLSEAMLTRANLEQADLSGARTTGARLDDADLRGATVDPVLWRTASLRGAKMEEEQRREYERARGGGGSRMRRDEILEEYRRGRRNFQHINLQEIELTNASLTGADLSYANLHHANLSRANLRSADLRNANLSHANLSGANLEEANLEAANLRGADLHEANLSGADLQEANLTQANLKDANLSDANLEQADLAGADLQGAVLDGANLHGANLNNANLSEAMLTRANLEQADLSGARTTGARLDDADLRGATVDPVLWRTASLRGAKMEEEQRREYERARGKSDDG

SEQ ID NO: 32 - protein, 1740 aa, Artificial Sequence
  SynRFR24.new_caps.x8.1 concatemer of eight beta solenoid domains, including N-terminal His tag
MGSSHHHHHHSSGLVPRGSRMRRDEILEEYRRGRRNFQHINLQEIELTNASLTGADLSYANLHHANLSRANLRSADLRNANLSHANLSGANLEEANLEAANLRGADLHEANLSGADLQEANLTQANLKDANLSDANLEQADLAGADLQGAVLDGANLHGANLNNANLSEAMLTRANLEQADLSGARTTGARLDDADLRGATVDPVLWRTASLRGAKMEEEQRREYERARGGGGSRMRRDEILEEYRRGRRNFQHINLQEIELTNASLTGADLSYANLHHANLSRANLRSADLRNANLSHANLSGANLEEANLEAANLRGADLHEANLSGADLQEANLTQANLKDANLSDANLEQADLAGADLQGAVLDGANLHGANLNNANLSEAMLTRANLEQADLSGARTTGARLDDADLRGATVDPVLWRTASLRGAKMEEEQRREYERARGGGGSRMRRDEILEEYRRGRRNFQHINLQEIELTNASLTGADLSYANLHHANLSRANLRSADLRNANLSHANLSGANLEEANLEAANLRGADLHEANLSGADLQEANLTQANLKDANLSDANLEQADLAGADLQGAVLDGANLHGANLNNANLSEAMLTRANLEQADLSGARTTGARLDDADLRGATVDPVLWRTASLRGAKMEEEQRREYERARGGGGSRMRRDEILEEYRRGRRNFQHINLQEIELTNASLTGADLSYANLHHANLSRANLRSADLRNANLSHANLSGANLEEANLEAANLRGADLHEANLSGADLQEANLTQANLKDANLSDANLEQADLAGADLQGAVLDGANLHGANLNNANLSEAMLTRANLEQADLSGARTTGARLDDADLRGATVDPVLWRTASLRGAKMEEEQRREYERARGGGGSRMRRDEILEEYRRGRRNFQHINLQEIELTNASLTGADLSYANLHHANLSRANLRSADLRNANLSHANLSGANLEEANLEAANLRGADLHEANLSGADLQEANLTQANLKDANLSDANLEQADLAGADLQGAVLDGANLHGANLNNANLSEAMLTRANLEQADLSGARTTGARLDDADLRGATVDPVLWRTASLRGAKMEEEQRREYERARGGGGSRMRRDEILEEYRRGRRNFQHINLQEIELTNASLTGADLSYANLHHANLSRANLRSADLRNANLSHANLSGANLEEANLEAANLRGADLHEANLSGADLQEANLTQANLKDANLSDANLEQADLAGADLQGAVLDGANLHGANLNNANLSEAMLTRANLEQADLSGARTTGARLDDADLRGATVDPVLWRTASLRGAKMEEEQRREYERARGGGGSRMRRDEILEEYRRGRRNFQHINLQEIELTNASLTGADLSYANLHHANLSRANLRSADLRNANLSHANLSGANLEEANLEAANLRGADLHEANLSGADLQEANLTQANLKDANLSDANLEQADLAGADLQGAVLDGANLHGANLNNANLSEAMLTRANLEQADLSGARTTGARLDDADLRGATVDPVLWRTASLRGAKMEEEQRREYERARGGGGSRMRRDEILEEYRRGRRNFQHINLQEIELTNASLTGADLSYANLHHANLSRANLRSADLRNANLSHANLSGANLEEANLEAANLRGADLHEANLSGADLQEANLTQANLKDANLSDANLEQADLAGADLQGAVLDGANLHGANLNNANLSEAMLTRANLEQADLSGARTTGARLDDADLRGATVDPVLWRTASLRGAKMEEEQRREYERARGKSDDG

SEQ ID NO: 33 - protein, 19 aa, Artificial Sequence
  His tag plus protease site
MGSSHHHHHHSSGLVPRGS

SEQ ID NO: 34 - protein, 4 aa, Artificial Sequence
  Linker sequence
GGGS

SEQ ID NO: 35 - DNA, 720 bp, Artificial Sequence
  SynRFT24.1 both capping sequences plus His tag
atgggtagcagccatcatcatcatcaccatagcagcggtctggttccgcgtggtagccacatgaatgttggtgaaattctgcgtcattatgcagcaggtaaacgcaattttcagcatattaacctgcaagaaattgaactgaccaatgcaagcctgaccggtgccgatctgagctatgcaaatctgcatcatgcaaatctgagccgtgccaatctgcgttctgcagacctgcgtaatgccaatctgtcacatgcgaatctgtcaggtgcaaatctggaagaagccaatctggaagccgctaatctgcgtggtgcggatctgcatgaagcgaatctgagtggcgctgatctgcaagaggcaaatctgacccaggcgaacctgaaagatgctaatctgtctgatgccaacctggaacaggcagatctggcaggggctgatctgcagggtgcagttctggacggtgctaatctgcatggcgcaaatctgaataatgcgaacctgagcgaagcaatgctgacccgtgcgaatctggagcaggccgacctgagcggtgcacgtaccaccggtgcacgtctggatgatgccgacctgcgtggtgcaaccgttgatccggttctgtggcgtaccgcaagcctggttggtgcacgtgttgatgttgatcaggcagttgcatttgcagcagcacatggtctgtgtctggcaggtggatccggctgctaa

SEQ ID NO: 36 - protein, 239 aa, Artificial Sequence
  synRFR24.2
MGSSHHHHHHSSGLVPRGSHMNVGEILRHYAAGKRNFQHINLQEIELTNASLTGADLSYANLHHANLSRANLRSADLRNANLSHANLSGANLEEANLEAANLRGADLHEANLSGADLQEANLTQANLKDANLSDANLEQADLAGADLQGAVLDGANLHGANLNNANLSEAMLTRANLEQADLSGARTTGARLDDASLHGATVDPVLWRTASLVGARVDVDQAVAFAAAHGLCLAGGSGC

SEQ ID NO: 37 - DNA, 720 bp, Artificial Sequence
  Nucleic acid encoding for synRFR24.2
atgggtagcagccatcatcatcatcaccatagcagcggtctggttccgcgtggtagccacatgaatgttggtgaaattctgcgtcattatgcagcaggtaaacgcaattttcagcatattaacctgcaagaaattgaactgaccaatgcaagcctgaccggtgccgatctgagctatgcaaatctgcatcatgcaaatctgagccgtgccaatctgcgttctgcagacctgcgtaatgccaatctgtcacatgcgaatctgtcaggtgcaaatctggaagaagccaatctggaagccgctaatctgcgtggtgcggatctgcatgaagcgaatctgagtggcgctgatctgcaagaggcaaatctgacccaggcgaacctgaaagatgctaatctgtctgatgccaacctggaacaggcagatctggcaggggctgatctgcagggtgcagttctggacggtgctaatctgcatggcgcaaatctgaataatgcgaacctgagcgaagcaatgctgacccgtgcgaatctggagcaggccgacctgagcggtgcacgtaccaccggtgcacgtctggatgatgctagcctccatggtgcaaccgttgatccggttctgtggcgtaccgcaagcctggttggtgcacgtgttgatgttgatcaggcagttgcatttgcagcagcacatggtctgtgtctggcaggtggatccggctgctaa

SEQ ID NO: 38 - protein, 219 aa, Artificial Sequence
  synRFR20.1
MGSSHHHHHHSSGLVPRGSHMNVGEILRHYAAGKRNFQHINLQEIELTNASLTGADLSYANLHHANLSRANLRSADLRNANLSHANLSGANLEEANLEAANLRGADLHEANLSGADLQEANLTQANLKDANLSDANLEQANLNNANLSEAMLTRANLEQADLSGARTTGARLDDADLRGATVDPVLWRTASLVGARVDVDQAVAFAAAHGLCLAGGSGC

SEQ ID NO: 39 - DNA, 660 bp, Artificial Sequence
  nucleic acid encoding synRFR20.1
atgggtagcagccatcatcatcatcaccatagcagcggtctggttccgcgtggtagccacatgaatgttggtgaaattctgcgtcattatgcagcaggtaaacgcaattttcagcatattaacctgcaagaaattgaactgaccaatgcaagcctgaccggtgccgatctgagctatgcaaatctgcatcatgcaaatctgagccgtgccaatctgcgttctgcagacctgcgtaatgccaatctgtcacatgcgaatctgtcaggtgcaaatctggaagaagccaatctggaagccgctaatctgcgtggtgcggatctgcatgaagcgaatctgagtggcgctgatctgcaagaggcaaatctgacccaggcgaacctgaaagatgctaatctgtctgatgccaacctggaacaggcaaatctgaataatgcgaacctgagcgaagcaatgctgacccgtgcgaatctggagcaggccgacctgagcggtgcacgtaccaccggtgcacgtctggatgatgccgacctgcgtggtgcaaccgttgatccggttctgtggcgtaccgcaagcctggttggtgcacgtgttgatgttgatcaggcagttgcatttgcagcagcacatggtctgtgtctggcaggtggatccggctgctaa

SEQ ID NO: 40 - protein, 259 aa, Artificial Sequence
  synRFR28.1
MGSSHHHHHHSSGLVPRGSHMNVGEILRHYAAGKRNFQHINLQEIELTNASLTGADLSYANLHHANLSRANLRSADLRNANLSHANLSGANLEEANLEAANLRGADLHEANLSGADLQEANLTQANLKDANLSDANLEQADLAGADLQGAVLDGANLHGADLNGADLKQADLSGADLGGANLNNANLSEAMLTRANLEQADLSGARTTGARLDDADLRGATVDPVLWRTASLVGARVDVDQAVAFAAAHGLCLAGGSGC

SEQ ID NO: 41 - DNA, 780 bp, Artificial Sequence
  nucleic acid encoding synRFR28.1
atgggtagcagccatcatcatcatcaccatagcagcggtctggttccgcgtggtagccacatgaatgttggtgaaattctgcgtcattatgcagcaggtaaacgcaattttcagcatattaacctgcaagaaattgaactgaccaatgcaagcctgaccggtgccgatctgagctatgcaaatctgcatcatgcaaatctgagccgtgccaatctgcgttctgcagacctgcgtaatgccaatctgtcacatgcgaatctgtcaggtgcaaatctggaagaagccaatctggaagccgctaatctgcgtggtgcggatctgcatgaagcgaatctgagtggcgctgatctgcaagaggcaaatctgacccaggcgaacctgaaagatgctaatctgtctgatgccaacctggaacaggcagatctggcaggggctgatctgcagggtgcagttctggacggtgctaatctgcatggcgcggacctcaacggtgccgatttaaaacaggctgatttatctggagcagatttaggtggcgcaaatctgaataatgcgaacctgagcgaagcaatgctgacccgtgcgaatctggagcaggccgacctgagcggtgcacgtaccaccggtgcacgtctggatgatgccgacctgcgtggtgcaaccgttgatccggttctgtggcgtaccgcaagcctggttggtgcacgtgttgatgttgatcaggcagttgcatttgcagcagcacatggtctgtgtctggcaggtggatccggctgctaa

SEQ ID NO: 42 - protein, 247 aa, Artificial Sequence
  synRFR24.t754
MGSSHHHHHHSSGLVPRGSHMNVGEILRHYAAGKRNFQHINLQEIELTNASLTGADLSYANLHHANLSRANLRSADLRNANLSHANLKGANLEEANLEAANLRGANLAGANLSGADLQEANLTQAQLGGWSDNGETGADLSDANLEQADLAGADLYGAVLDGANLHGANLNNANLDNAMLTRANLEQADLSGARTTGARLDDADLRGATVDPVLWRTASLVGARVDVDQAVAFAAAHGLCLAGGSGC

SEQ ID NO: 43 - DNA, 744 bp, Artificial Sequence
  nucleic acid encoding synRFR24.t754
atgggtagcagccatcatcatcatcaccatagcagcggtctggttccgcgtggtagccacatgaatgttggtgaaattctgcgtcattatgcagcaggtaaacgcaattttcagcatattaacctgcaagaaattgaactgaccaatgcaagcctgaccggtgccgatctgagctatgcaaatctgcatcatgcaaatctgagccgtgccaatctgcgttctgcagacctgcgtaatgccaatctgtcacatgcgaatctgaaaggtgcaaatctggaagaagccaatctggaagccgctaatctgcgtggtgcgaacctggcgggcgcgaatctgagtggcgctgatctgcaagaggcaaatctgacccaggcgcagctgggcggctggagcgataacggcgaaaccggcgctgatctgtctgatgccaacctggaacaggcagatctggcaggggctgatctgtatggtgcagttctggacggtgctaatctgcatggcgcaaatctgaataatgcgaacctggataacgcaatgctgacccgtgcgaatctggagcaggccgacctgagcggtgcacgtaccaccggtgcacgtctggatgatgccgacctgcgtggtgcaaccgttgatccggttctgtggcgtaccgcaagcctggttggtgcacgtgttgatgttgatcaggcagttgcatttgcagcagcacatggtctgtgtctggcaggtggatccggctgctaa

SEQ ID NO: 44 - protein, 247 aa, Artificial Sequence
  synRFR24.t801
MGSSHHHHHHSSGLVPRGSHMNVGEILRHYAAGKRNFQHINLQEIELTNASLTGADLSYANLHHANLSRANLRSADLRNANLSHANLRGANLEEANLEAANLRGADLIGANLSGADLQEANLTQAQLGLGVEDGGLGADLSDANLEQADLAGANLAGAVLDGANLHGANLNNANLDYAMLTRANLEQADLSGARTTGARLDDADLRGATVDPVLWRTASLVGARVDVDQAVAFAAAHGLCLAGGSGC

SEQ ID NO: 45 - DNA, 744 bp, Artificial Sequence
  Nucleic acid encoding synRFR24.t801
atgggtagcagccatcatcatcatcaccatagcagcggtctggttccgcgtggtagccacatgaatgttggtgaaattctgcgtcattatgcagcaggtaaacgcaattttcagcatattaacctgcaagaaattgaactgaccaatgcaagcctgaccggtgccgatctgagctatgcaaatctgcatcatgcaaatctgagccgtgccaatctgcgttctgcagacctgcgtaatgccaatctgtcacatgcgaatctgcgcggtgcaaatctggaagaagccaatctggaagccgctaatctgcgtggtgcggatctgattggcgcgaatctgagtggcgctgatctgcaagaggcaaatctgacccaggcgcagctgggcctgggcgtggaagatggcggcctgggcgctgatctgtctgatgccaacctggaacaggcagatctggcaggggctaacctggcgggtgcagttctggacggtgctaatctgcatggcgcaaatctgaataatgcgaacctggattatgcaatgctgacccgtgcgaatctggagcaggccgacctgagcggtgcacgtaccaccggtgcacgtctggatgatgccgacctgcgtggtgcaaccgttgatccggttctgtggcgtaccgcaagcctggttggtgcacgtgttgatgttgatcaggcagttgcatttgcagcagcacatggtctgtgtctggcaggtggatccggctgctaa

SEQ ID NO: 46 - protein, 247 aa, Artificial Sequence
  synRFR24. t1117
MGSSHHHHHHSSGLVPRGSHMNVGEILRHYAAGKRNFQHINLQEIELTNASLTGADLSYANLHHANLSRANLRSADLRNANLSHANLRGANLEEANLEAANLRGADLVGANLSGADLQEANLTQAQLGGVYRLGEPGADLSDANLEQADLAGANLMGAVLDGANLHGANLNNANLDYAMLTRANLEQADLSGARTTGARLDDADLRGATVDPVLWRTASLVGARVDVDQAVAFAAAHGLCLAGGSGC

SEQ ID NO: 47 - DNA, 744 bp, Artificial Sequence
  nucleic acid encoding synRFR24. t1117
atgggtagcagccatcatcatcatcaccatagcagcggtctggttccgcgtggtagccacatgaatgttggtgaaattctgcgtcattatgcagcaggtaaacgcaattttcagcatattaacctgcaagaaattgaactgaccaatgcaagcctgaccggtgccgatctgagctatgcaaatctgcatcatgcaaatctgagccgtgccaatctgcgttctgcagacctgcgtaatgccaatctgtcacatgcgaatctgcgcggtgcaaatctggaagaagccaatctggaagccgctaatctgcgtggtgcggatctggtgggcgcgaatctgagtggcgctgatctgcaagaggcaaatctgacccaggcgcagctgggcggcgtgtatcgcctgggcgaaccgggcgctgatctgtctgatgccaacctggaacaggcagatctggcaggggctaacctgatgggtgcagttctggacggtgctaatctgcatggcgcaaatctgaataatgcgaacctggattatgcaatgctgacccgtgcgaatctggagcaggccgacctgagcggtgcacgtaccaccggtgcacgtctggatgatgccgacctgcgtggtgcaaccgttgatccggttctgtggcgtaccgcaagcctggttggtgcacgtgttgatgttgatcaggcagttgcatttgcagcagcacatggtctgtgtctggcaggtggatccggctgctaa

SEQ ID NO: 48 - protein, 247 aa, Artificial Sequence
  synRFR24.t1166
MGSSHHHHHHSSGLVPRGSHMNVGEILRHYAAGKRNFQHINLQEIELTNASLTGADLSYANLHHANLSRANLRSADLRNANLSHANLSGANLEEANLEAANLRGADLRGANLSGADLQEANLTQAKLGTWSSSGLTGADLSDANLEQADLAGADLKGAVLDGANLHGANLNNANLDYAMLTRANLEQADLSGARTTGARLDDADLRGATVDPVLWRTASLVGARVDVDQAVAFAAAHGLCLAGGSGC

SEQ ID NO: 49 - DNA, 744 bp, Artificial Sequence
  nucleic acid encoding synRFR24.t1166
atgggtagcagccatcatcatcatcaccatagcagcggtctggttccgcgtggtagccacatgaatgttggtgaaattctgcgtcattatgcagcaggtaaacgcaattttcagcatattaacctgcaagaaattgaactgaccaatgcaagcctgaccggtgccgatctgagctatgcaaatctgcatcatgcaaatctgagccgtgccaatctgcgttctgcagacctgcgtaatgccaatctgtcacatgcgaatctgtcaggtgcaaatctggaagaagccaatctggaagccgctaatctgcgtggtgcggatctgcgcggcgcgaatctgagtggcgctgatctgcaagaggcaaatctgacccaggcgaaactgggcacctggagcagcagcggcctgaccggcgctgatctgtctgatgccaacctggaacaggcagatctggcaggggctgatctgaaaggtgcagttctggacggtgctaatctgcatggcgcaaatctgaataatgcgaacctggattatgcaatgctgacccgtgcgaatctggagcaggccgacctgagcggtgcacgtaccaccggtgcacgtctggatgatgccgacctgcgtggtgcaaccgttgatccggttctgtggcgtaccgcaagcctggttggtgcacgtgttgatgttgatcaggcagttgcatttgcagcagcacatggtctgtgtctggcaggtggatccggctgctaa

SEQ ID NO: 50 - protein, 247 aa, Artificial Sequence
  synRFR24.t1428
MGSSHHHHHHSSGLVPRGSHMNVGEILRHYAAGKRNFQHINLQEIELTNASLTGADLSYANLHHANLSRANLRSADLRNANLSHANLSGANLEEANLEAANLRGANLVGANLSGADLQEANLTQAMLGQTYPWGTVGADLSDANLEQADLAGAQLVGAVLDGANLHGANLNNANLDNAMLTRANLEQADLSGARTTGARLDDADLRGATVDPVLWRTASLVGARVDVDQAVAFAAAHGLCLAGGSGC

SEQ ID NO: 51 - DNA, 744 bp, Artificial Sequence
  nucleic acid encoding synRFR24.t1428
atgggtagcagccatcatcatcatcaccatagcagcggtctggttccgcgtggtagccacatgaatgttggtgaaattctgcgtcattatgcagcaggtaaacgcaattttcagcatattaacctgcaagaaattgaactgaccaatgcaagcctgaccggtgccgatctgagctatgcaaatctgcatcatgcaaatctgagccgtgccaatctgcgttctgcagacctgcgtaatgccaatctgtcacatgcgaatctgtcaggtgcaaatctggaagaagccaatctggaagccgctaatctgcgtggtgcgaacctggtgggcgcgaatctgagtggcgctgatctgcaagaggcaaatctgacccaggcgatgctgggccagacctatccgtggggcaccgtgggcgctgatctgtctgatgccaacctggaacaggcagatctggcaggggctcagctggtgggtgcagttctggacggtgctaatctgcatggcgcaaatctgaataatgcgaacctggataacgcaatgctgacccgtgcgaatctggagcaggccgacctgagcggtgcacgtaccaccggtgcacgtctggatgatgccgacctgcgtggtgcaaccgttgatccggttctgtggcgtaccgcaagcctggttggtgcacgtgttgatgttgatcaggcagttgcatttgcagcagcacatggtctgtgtctggcaggtggatccggctgctaa

SEQ ID NO: 52 - protein, 247 aa, Artificial Sequence
  synRFR24.t1555
MGSSHHHHHHSSGLVPRGSHMNVGEILRHYAAGKRNFQHINLQEIELTNASLTGADLSYANLHHANLSRANLRSADLRNANLSHANLSGANLEEANLEAANLRGADLAGANLSGADLQEANLTQAMLGKDEDGVVYGADLSDANLEQADLAGAQLVGAVLDGANLHGANLNNANLDNAMLTRANLEQADLSGARTTGARLDDADLRGATVDPVLWRTASLVGARVDVDQAVAFAAAHGLCLAGGSGC

SEQ ID NO: 53 - DNA, 744 bp, Artificial Sequence
  nucleic acid encoding synRFR24.t1555
atgggtagcagccatcatcatcatcaccatagcagcggtctggttccgcgtggtagccacatgaatgttggtgaaattctgcgtcattatgcagcaggtaaacgcaattttcagcatattaacctgcaagaaattgaactgaccaatgcaagcctgaccggtgccgatctgagctatgcaaatctgcatcatgcaaatctgagccgtgccaatctgcgttctgcagacctgcgtaatgccaatctgtcacatgcgaatctgtcaggtgcaaatctggaagaagccaatctggaagccgctaatctgcgtggtgcggatctggcgggcgcgaatctgagtggcgctgatctgcaagaggcaaatctgacccaggcgatgctgggcaaagatgaagatggcgtggtgtatggcgctgatctgtctgatgccaacctggaacaggcagatctggcaggggctcagctggtgggtgcagttctggacggtgctaatctgcatggcgcaaatctgaataatgcgaacctggataacgcaatgctgacccgtgcgaatctggagcaggccgacctgagcggtgcacgtaccaccggtgcacgtctggatgatgccgacctgcgtggtgcaaccgttgatccggttctgtggcgtaccgcaagcctggttggtgcacgtgttgatgttgatcaggcagttgcatttgcagcagcacatggtctgtgtctggcaggtggatccggctgctaa

SEQ ID NO: 54 - protein, 247 aa, Artificial Sequence
  synRFR24.t1916
MGSSHHHHHHSSGLVPRGSHMNVGEILRHYAAGKRNFQHINLQEIELTNASLTGADLSYANLHHANLSRANLRSADLRNANLSHANLSGANLEEANLEAANLRGALLTGANLSGADLQEANLTQAWLGRDPRLGLSGADLSDANLEQADLAGAQLKGAVLDGANLHGANLNNANLDNAMLTRANLEQADLSGARTTGARLDDADLRGATVDPVLWRTASLVGARVDVDQAVAFAAAHGLCLAGGSGC

SEQ ID NO: 55 - DNA, 744 bp, Artificial Sequence
  nucleic acid encoding synRFR24.t1916
atgggtagcagccatcatcatcatcaccatagcagcggtctggttccgcgtggtagccacatgaatgttggtgaaattctgcgtcattatgcagcaggtaaacgcaattttcagcatattaacctgcaagaaattgaactgaccaatgcaagcctgaccggtgccgatctgagctatgcaaatctgcatcatgcaaatctgagccgtgccaatctgcgttctgcagacctgcgtaatgccaatctgtcacatgcgaatctgtcaggtgcaaatctggaagaagccaatctggaagccgctaatctgcgtggtgcgctgctgaccggcgcgaatctgagtggcgctgatctgcaagaggcaaatctgacccaggcgtggctgggccgcgatccgcgcctgggcctgagcggcgctgatctgtctgatgccaacctggaacaggcagatctggcaggggctcagctgaaaggtgcagttctggacggtgctaatctgcatggcgcaaatctgaataatgcgaacctggataacgcaatgctgacccgtgcgaatctggagcaggccgacctgagcggtgcacgtaccaccggtgcacgtctggatgatgccgacctgcgtggtgcaaccgttgatccggttctgtggcgtaccgcaagcctggttggtgcacgtgttgatgttgatcaggcagttgcatttgcagcagcacatggtctgtgtctggcaggtggatccggctgctaa

SEQ ID NO: 56 - protein, 247 aa, Artificial Sequence
  synRFR24.t2570
MGSSHHHHHHSSGLVPRGSHMNVGEILRHYAAGKRNFQHINLQEIELTNASLTGADLSYANLHHANLSRANLRSADLRNANLSHANLKGANLEEANLEAANLRGANLAGANLSGADLQEANLTQADLGGPPDEGKTGADLSDANLEQADLAGAQLYGAVLDGANLHGANLNNANLDYAMLTRANLEQADLSGARTTGARLDDADLRGATVDPVLWRTASLVGARVDVDQAVAFAAAHGLCLAGGSGC

SEQ ID NO: 57 - DNA, 744 bp, Artificial Sequence
  nucleic acid encoding synRFR24.t2570
atgggtagcagccatcatcatcatcaccatagcagcggtctggttccgcgtggtagccacatgaatgttggtgaaattctgcgtcattatgcagcaggtaaacgcaattttcagcatattaacctgcaagaaattgaactgaccaatgcaagcctgaccggtgccgatctgagctatgcaaatctgcatcatgcaaatctgagccgtgccaatctgcgttctgcagacctgcgtaatgccaatctgtcacatgcgaatctgaaaggtgcaaatctggaagaagccaatctggaagccgctaatctgcgtggtgcgaacctggcgggcgcgaatctgagtggcgctgatctgcaagaggcaaatctgacccaggcggatctgggcggcccgccggatgaaggcaaaaccggcgctgatctgtctgatgccaacctggaacaggcagatctggcaggggctcagctgtatggtgcagttctggacggtgctaatctgcatggcgcaaatctgaataatgcgaacctggattatgcaatgctgacccgtgcgaatctggagcaggccgacctgagcggtgcacgtaccaccggtgcacgtctggatgatgccgacctgcgtggtgcaaccgttgatccggttctgtggcgtaccgcaagcctggttggtgcacgtgttgatgttgatcaggcagttgcatttgcagcagcacatggtctgtgtctggcaggtggatccggctgctaa

SEQ ID NO: 58 - protein, 247 aa, Artificial Sequence
  synRFR24.t3280
MGSSHHHHHHSSGLVPRGSHMNVGEILRHYAAGKRNFQHINLQEIELTNASLTGADLSYANLHHANLSRANLRSADLRNANLSHANLSGANLEEANLEAANLRGADLRGANLSGADLQEANLTQAKLGGYDDEGLGGADLSDANLEQADLAGAELFGAVLDGANLHGANLNNANLDKAMLTRANLEQADLSGARTTGARLDDADLRGATVDPVLWRTASLVGARVDVDQAVAFAAAHGLCLAGGSGC

SEQ ID NO: 59 - DNA, 744 bp, Artificial Sequence
  nucleic acid encoding synRFR24.t3280
atgggtagcagccatcatcatcatcaccatagcagcggtctggttccgcgtggtagccacatgaatgttggtgaaattctgcgtcattatgcagcaggtaaacgcaattttcagcatattaacctgcaagaaattgaactgaccaatgcaagcctgaccggtgccgatctgagctatgcaaatctgcatcatgcaaatctgagccgtgccaatctgcgttctgcagacctgcgtaatgccaatctgtcacatgcgaatctgagcggtgcaaatctggaagaagccaatctggaagccgctaatctgcgtggtgcggatctgcgcggcgcgaatctgagtggcgctgatctgcaagaggcaaatctgacccaggcgaaactgggcggctatgatgatgaaggcctgggcggcgctgatctgtctgatgccaacctggaacaggcagatctggcaggggctgaactgtttggtgcagttctggacggtgctaatctgcatggcgcaaatctgaataatgcgaacctggataaagcaatgctgacccgtgcgaatctggagcaggccgacctgagcggtgcacgtaccaccggtgcacgtctggatgatgccgacctgcgtggtgcaaccgttgatccggttctgtggcgtaccgcaagcctggttggtgcacgtgttgatgttgatcaggcagttgcatttgcagcagcacatggtctgtgtctggcaggtggatccggctgctaa

SEQ ID NO: 60 - protein, 247 aa, Artificial Sequence
  synRFR24.t3284
MGSSHHHHHHSSGLVPRGSHMNVGEILRHYAAGKRNFQHINLQEIELTNASLTGADLSYANLHHANLSRANLRSADLRNANLSHANLEGANLEEANLEAANLRGARLAGANLSGADLQEANLTQANLGGPPDDGDPGADLSDANLEQADLAGANLAGAVLDGANLHGANLNNANLDNAMLTRANLEQADLSGARTTGARLDDADLRGATVDPVLWRTASLVGARVDVDQAVAFAAAHGLCLAGGSGC

SEQ ID NO: 61 - DNA, 744 bp, Artificial Sequence
  nucleic acid encoding synRFR24.t3284
atgggtagcagccatcatcatcatcaccatagcagcggtctggttccgcgtggtagccacatgaatgttggtgaaattctgcgtcattatgcagcaggtaaacgcaattttcagcatattaacctgcaagaaattgaactgaccaatgcaagcctgaccggtgccgatctgagctatgcaaatctgcatcatgcaaatctgagccgtgccaatctgcgttctgcagacctgcgtaatgccaatctgtcacatgcgaatctggaaggtgcaaatctggaagaagccaatctggaagccgctaatctgcgtggtgcgcgcctggcgggcgcgaatctgagtggcgctgatctgcaagaggcaaatctgacccaggcgaacctgggcggcccgccggatgatggcgatccgggcgctgatctgtctgatgccaacctggaacaggcagatctggcaggggctaacctggcgggtgcagttctggacggtgctaatctgcatggcgcaaatctgaataatgcgaacctggataacgcaatgctgacccgtgcgaatctggagcaggccgacctgagcggtgcacgtaccaccggtgcacgtctggatgatgccgacctgcgtggtgcaaccgttgatccggttctgtggcgtaccgcaagcctggttggtgcacgtgttgatgttgatcaggcagttgcatttgcagcagcacatggtctgtgtctggcaggtggatccggctgctaa

SEQ ID NO: 62 - protein, 493 aa, Artificial Sequence
  synRFR24.t1428 sfGFP
MGSSHHHHHHSSGLVPRGSHMNVGEILRHYAAGKRNFQHINLQEIELTNASLTGADLSYANLHHANLSRANLRSADLRNANLSHANLSGANLEEANLEAANLRGANLVGANLSGADLQEANLTQAMLGQTYPGGGGSMRKGEELFTGVVPILVELDGDVNGHKFSVRGEGEGDATNGKLTLKFICTTGKLPVPWPTLVTTLTYGVQCFARYPDHMKQHDFFKSAMPEGYVQERTISFKDDGTYKTRAEVKFEGDTLVNRIELKGIDFKEDGNILGHKLEYNFNSHNVYITADKQKNGIKANFKIRHNVEDGSVQLADHYQQNTPIGDGPVLLPDNHYLSTQSVLSKDPNEKRDHMVLLEFVTAAGITHGMDELSGGGGWGTVGADLSDANLEQADLAGAQLVGAVLDGANLHGANLNNANLDNAMLTRANLEQADLSGARTTGARLDDADLRGATVDPVLWRTASLVGARVDVDQAVAFAAAHGLCLAGGSGC

SEQ ID NO: 63 - DNA, 1482 bp, Artificial Sequence
  nucleic acid encoding synRFR24.t1428 sfGFP
atgggtagcagccatcatcatcatcaccatagcagcggtctggttccgcgtggtagccacatgaatgttggtgaaattctgcgtcattatgcagcaggtaaacgcaattttcagcatattaacctgcaagaaattgaactgaccaatgcaagcctgaccggtgccgatctgagctatgcaaatctgcatcatgcaaatctgagccgtgccaatctgcgttctgcagacctgcgtaatgccaatctgtcacatgcgaatctgtcaggtgcaaatctggaagaagccaatctggaagccgctaatctgcgtggtgcgaacctggtgggcgcgaatctgagtggcgctgatctgcaagaggcaaatctgacccaggcgatgctgggccagacctatccgggaggtggaggctcaatgcgtaaaggcgaagagctgttcactggtgtcgtccctattctggtggaactggatggtgatgtcaacggtcataagttttccgtgcgtggcgagggtgaaggtgacgcaactaatggtaaactgacgctgaagttcatctgtactactggtaaactgccggtaccttggccgactctggtaacgacgctgacttatggtgttcagtgctttgctcgttatccggaccatatgaagcagcatgacttcttcaagtccgccatgccggaaggctatgtgcaggaacgcacgatttcctttaaggatgacggcacgtacaaaacgcgtgcggaagtgaaatttgaaggcgataccctggtaaaccgcattgagctgaaaggcattgactttaaagaagacggcaatatcctgggccataagctggaatacaattttaacagccacaatgtttacatcaccgccgataaacaaaaaaatggcattaaagcgaattttaaaattcgccacaacgtggaggatggcagcgtgcagctggctgatcactaccagcaaaacactccaatcggtgatggtcctgttctgctgccagacaatcactatctgagcacgcaaagcgttctgtctaaagatccgaacgagaaacgcgatcatatggttctgctggagttcgtaaccgcagcgggcatcacgcatggtatggatgaactgtctggaggcggtggatggggcaccgtgggcgctgatctgtctgatgccaacctggaacaggcagatctggcaggggctcagctggtgggtgcagttctggacggtgctaatctgcatggcgcaaatctgaataatgcgaacctggataacgcaatgctgacccgtgcgaatctggagcaggccgacctgagcggtgcacgtaccaccggtgcacgtctggatgatgccgacctgcgtggtgcaaccgttgatccggttctgtggcgtaccgcaagcctggttggtgcacgtgttgatgttgatcaggcagttgcatttgcagcagcacatggtctgtgtctggcaggtggatccggctgctaa

SEQ ID NO: 64 - protein, 493 aa, Artificial Sequence
  synRFR24.t1428 sfGFPmut
MGSSHHHHHHSSGLVPRGSHMNVGEILRHYAAGKRNFQHINLQEIELTNASLTGADLSYANLHHANLSRANLRSADLRNANLSHANLSGANLEEANLEAANLRGANLVGANLSGADLQEANLTQAMLGQTYPGGGGSMRKGEELFTGVVPILVELDGDVNGHKFSVRGEGEGDATNGKLTLKFICTTGKLPVPWPTLVTTLTYGVQCFARYPDHMKQHDFFKSAMPEGYVQERTISFKDDGTYKTRAEVKFEGDTLVNRIELKGIDFKEDGNILGHKLEYNFNSHNVYITADKQKNGIKANFKIRHNVEDGSVQLADHYQQNTPIGDGPVLLPDNHYLSTQSVLSKDPNEKRDHMVLLEFVTAAGITHGMDELSGGGGAGTVGADLSDANLEQADLAGAQLVGAVLDGANLHGANLNNANLDNAMLTRANLEQADLSGARTTGARLDDADLRGATVDPVLWRTASLVGARVDVDQAVAFAAAHGLCLAGGSGC

SEQ ID NO: 65 - DNA, 1482 bp, Artificial Sequence
  nucleic acid encoding synRFR24.t1428 sfGFPmut
atgggtagcagccatcatcatcatcaccatagcagcggtctggttccgcgtggtagccacatgaatgttggtgaaattctgcgtcattatgcagcaggtaaacgcaattttcagcatattaacctgcaagaaattgaactgaccaatgcaagcctgaccggtgccgatctgagctatgcaaatctgcatcatgcaaatctgagccgtgccaatctgcgttctgcagacctgcgtaatgccaatctgtcacatgcgaatctgtcaggtgcaaatctggaagaagccaatctggaagccgctaatctgcgtggtgcgaacctggtgggcgcgaatctgagtggcgctgatctgcaagaggcaaatctgacccaggcgatgctgggccagacctatccgggaggtggaggctcaatgcgtaaaggcgaagagctgttcactggtgtcgtccctattctggtggaactggatggtgatgtcaacggtcataagttttccgtgcgtggcgagggtgaaggtgacgcaactaatggtaaactgacgctgaagttcatctgtactactggtaaactgccggtaccttggccgactctggtaacgacgctgacttatggtgttcagtgctttgctcgttatccggaccatatgaagcagcatgacttcttcaagtccgccatgccggaaggctatgtgcaggaacgcacgatttcctttaaggatgacggcacgtacaaaacgcgtgcggaagtgaaatttgaaggcgataccctggtaaaccgcattgagctgaaaggcattgactttaaagaagacggcaatatcctgggccataagctggaatacaattttaacagccacaatgtttacatcaccgccgataaacaaaaaaatggcattaaagcgaattttaaaattcgccacaacgtggaggatggcagcgtgcagctggctgatcactaccagcaaaacactccaatcggtgatggtcctgttctgctgccagacaatcactatctgagcacgcaaagcgttctgtctaaagatccgaacgagaaacgcgatcatatggttctgctggagttcgtaaccgcagcgggcatcacgcatggtatggatgaactgtctggaggcggtggagctggcaccgtgggcgctgatctgtctgatgccaacctggaacaggcagatctggcaggggctcagctggtgggtgcagttctggacggtgctaatctgcatggcgcaaatctgaataatgcgaacctggataacgcaatgctgacccgtgcgaatctggagcaggccgacctgagcggtgcacgtaccaccggtgcacgtctggatgatgccgacctgcgtggtgcaaccgttgatccggttctgtggcgtaccgcaagcctggttggtgcacgtgttgatgttgatcaggcagttgcatttgcagcagcacatggtctgtgtctggcaggtggatccggctgctaa

SEQ ID NO: 66 - protein, 120 aa, Artificial Sequence
  Solenoid domain sequence of synRFR24.2
ANLHHANLSRANLRSADLRNANLSHANLSGANLEEANLEAANLRGADLHEANLSGADLQEANLTQANLKDANLSDANLEQADLAGADLQGAVLDGANLHGANLNNANLSEAMLTRANLEQ

SEQ ID NO: 67 - protein, 100 aa, Artificial Sequence
  Solenoid domain sequence of synRFR20.1
ANLHHANLSRANLRSADLRNANLSHANLSGANLEEANLEAANLRGADLHEANLSGADLQEANLTQANLKDANLSDANLEQANLNNANLSEAMLTRANLEQ

SEQ ID NO: 68 - protein, 140 aa, Artificial Sequence
  Solenoid domain sequence of synRFR28.1
ANLHHANLSRANLRSADLRNANLSHANLSGANLEEANLEAANLRGADLHEANLSGADLQEANLTQANLKDANLSDANLEQADLAGADLQGAVLDGANLHGADLNGADLKQADLSGADLGGANLNNANLSEAMLTRANLEQ

SEQ ID NO: 69 - protein, 128 aa, Artificial Sequence
  Solenoid domain sequence of synRFR24.t764
ANLHHANLSRANLRSADLRNANLSHANLKGANLEEANLEAANLRGANLAGANLSGADLQEANLTQAQLGGWSDNGETGADLSDANLEQADLAGADLYGAVLDGANLHGANLNNANLDNAMLTRANLEQ

SEQ ID NO: 70 - protein, 128 aa, Artificial Sequence
  Solenoid domain sequence of synRFR24.t801
ANLHHANLSRANLRSADLRNANLSHANLRGANLEEANLEAANLRGADLIGANLSGADLQEANLTQAQLGLGVEDGGLGADLSDANLEQADLAGANLAGAVLDGANLHGANLNNANLDYAMLTRANLEQ

SEQ ID NO: 71 - protein, 128 aa, Artificial Sequence
  Solenoid domain sequence of synRFR24.t1117
ANLHHANLSRANLRSADLRNANLSHANLRGANLEEANLEAANLRGADLVGANLSGADLQEANLTQAQLGGVYRLGEPGADLSDANLEQADLAGANLMGAVLDGANLHGANLNNANLDYAMLTRANLEQ

SEQ ID NO: 72 - protein, 128 aa, Artificial Sequence
  Solenoid domain sequence of synRFR24.t1166
ANLHHANLSRANLRSADLRNANLSHANLSGANLEEANLEAANLRGADLRGANLSGADLQEANLTQAKLGTWSSSGLTGADLSDANLEQADLAGADLKGAVLDGANLHGANLNNANLDYAMLTRANLEQ

SEQ ID NO: 73 - protein, 128 aa, Artificial Sequence
  Solenoid domain sequence of synRFR24.t1428
ANLHHANLSRANLRSADLRNANLSHANLSGANLEEANLEAANLRGANLVGANLSGADLQEANLTQAMLGQTYPWGTVGADLSDANLEQADLAGAQLVGAVLDGANLHGANLNNANLDNAMLTRANLEQ

SEQ ID NO: 74 - protein, 128 aa, Artificial Sequence
  Solenoid domain sequence of synRFR24.t1555
ANLHHANLSRANLRSADLRNANLSHANLSGANLEEANLEAANLRGADLAGANLSGADLQEANLTQAMLGKDEDGVVYGADLSDANLEQADLAGAQLVGAVLDGANLHGANLNNANLDNAMLTRANLEQ

SEQ ID NO: 75 - protein, 128 aa, Artificial Sequence
  Solenoid domain sequence of synRFR24.t1916
ANLHHANLSRANLRSADLRNANLSHANLSGANLEEANLEAANLRGALLTGANLSGADLQEANLTQAWLGRDPRLGLSGADLSDANLEQADLAGAQLKGAVLDGANLHGANLNNANLDNAMLTRANLEQ

SEQ ID NO: 76 - protein, 128 aa, Artificial Sequence
  Solenoid domain sequence of synRFR24.t2570
ANLHHANLSRANLRSADLRNANLSHANLKGANLEEANLEAANLRGANLAGANLSGADLQEANLTQADLGGPPDEGKTGADLSDANLEQADLAGAQLYGAVLDGANLHGANLNNANLDYAMLTRANLEQ

SEQ ID NO: 77 - protein, 128 aa, Artificial Sequence
  Solenoid domain sequence of synRFR24.t3280
ANLHHANLSRANLRSADLRNANLSHANLSGANLEEANLEAANLRGADLRGANLSGADLQEANLTQAKLGGYDDEGLGGADLSDANLEQADLAGAELFGAVLDGANLHGANLNNANLDKAMLTRANLEQ

SEQ ID NO: 78 - protein, 128 aa, Artificial Sequence
  Solenoid domain sequence of synRFR24.t3284
ANLHHANLSRANLRSADLRNANLSHANLEGANLEEANLEAANLRGARLAGANLSGADLQEANLTQANLGGPPDDGDPGADLSDANLEQADLAGANLAGAVLDGANLHGANLNNANLDNAMLTRANLEQ

SEQ ID NO: 79 - protein, 374 aa, Artificial Sequence
  Solenoid domain sequence of synRFR24.t1428.sfGFP
ANLHHANLSRANLRSADLRNANLSHANLSGANLEEANLEAANLRGANLVGANLSGADLQEANLTQAMLGQTYPGGGGSMRKGEELFTGVVPILVELDGDVNGHKFSVRGEGEGDATNGKLTLKFICTTGKLPVPWPTLVTTLTYGVQCFARYPDHMKQHDFFKSAMPEGYVQERTISFKDDGTYKTRAEVKFEGDTLVNRIELKGIDFKEDGNILGHKLEYNFNSHNVYITADKQKNGIKANFKIRHNVEDGSVQLADHYQQNTPIGDGPVLLPDNHYLSTQSVLSKDPNEKRDHMVLLEFVTAAGITHGMDELSGGGGWGTVGADLSDANLEQADLAGAQLVGAVLDGANLHGANLNNANLDNAMLTRANLEQ

SEQ ID NO: 80 - protein, 374 aa, Artificial Sequence
  Solenoid domain sequence of synRFR24.t1428.sfGFP
ANLHHANLSRANLRSADLRNANLSHANLSGANLEEANLEAANLRGANLVGANLSGADLQEANLTQAMLGQTYPGGGGSMRKGEELFTGVVPILVELDGDVNGHKFSVRGEGEGDATNGKLTLKFICTTGKLPVPWPTLVTTLTYGVQCFARYPDHMKQHDFFKSAMPEGYVQERTISFKDDGTYKTRAEVKFEGDTLVNRIELKGIDFKEDGNILGHKLEYNFNSHNVYITADKQKNGIKANFKIRHNVEDGSVQLADHYQQNTPIGDGPVLLPDNHYLSTQSVLSKDPNEKRDHMVLLEFVTAAGITHGMDELSGGGGAGTVGADLSDANLEQADLAGAQLVGAVLDGANLHGANLNNANLDNAMLTRANLEQ

SEQ ID NO: 81 - protein, 5 aa, Artificial Sequence
  Tail sequence
KSDDG

SEQ ID NO: 82 - protein, 30 aa, Artificial Sequence
  N-terminal capping consensus sequence
  VARIANT join(1,3..6,9..10,12..13,15..17,19..20,22,24..25,27,29..30): Wherein Xaa is any amino acid
  VARIANT 26: Wherein Xaa is Ile or Ala
XMXXXXILXXYXXGXXXFXXIXLXXXXLXX

SEQ ID NO: 83 - protein, 46 aa, Artificial Sequence
  C-terminal capping consensus sequence
  VARIANT join(2,4..5,7,9..10,12,14..15,17,19,24..25,27,29,32,34..40,42..43,45..46): Wherein Xaa is any amino acid
  VARIANT 3: Wherein Xaa is Thr, Leu or Phe
  VARIANT 8: Wherein Xaa is Leu or Phe
  VARIANT 13: Wherein Xaa is Leu or Phe
  VARIANT 33: Wherein Xaa is Met or Val
  VARIANT 41: Wherein Xaa is Tyr or Phe
AXXXXAXXXXAXXXXAXVXPVLWXXAXLXGAXXXXXXXXXXXXAXX

SEQ ID NO: 84 - protein, 30 aa, Artificial Sequence
  rfr_ref_minprep_ren_neg_num_20_0004.pdb NCAP
SMGKNEILNQYKNGRHDFSGINLAKADLEN

SEQ ID NO: 85 - protein, 30 aa, Artificial Sequence
  rfr_ref_minprep_ren_neg_num_21_0003.pdb NCAP
TMQTKQILKEYKKGRTNFSGINLANANLKN

SEQ ID NO: 86 - protein, 30 aa, Artificial Sequence
  rfr_ref_minprep_ren_neg_num_22_0001.pdb NCAP
TMRTKDILKQYNNGRHNFSGIDLANADLEK

SEQ ID NO: 87 - protein, 30 aa, Artificial Sequence
  rfr_ref_minprep_ren_neg_num_23_0004.pdb
TMQTNQILKEYKNGRHNFSKINLANANLQN

SEQ ID NO: 88 - protein, 30 aa, Artificial Sequence
  rfr_ref_minprep_ren_neg_num_24_0002.pdb NCAP
SMGTKEILNEYKKGRKKFANINLANADLSN

SEQ ID NO: 89 - protein, 30 aa, Artificial Sequence
  rfr_ref_minprep_ren_neg_num_25_0003.pdb NCAP
TMRRDDILREYNNGRHNFSGINLAKADLRD

SEQ ID NO: 90 - protein, 30 aa, Artificial Sequence
  rfr_ref_minprep_ren_neg_num_26_0004.pdb NCAP
NMKTNKILKNYKKGRHDFTGIDLANADLEN

SEQ ID NO: 91 - protein, 30 aa, Artificial Sequence
  rfr_ref_minprep_ren_neg_num_27_0004.pdb NCAP
SMQADQILQQYDNGRRNFSGIDLENADLRN

SEQ ID NO: 92 - protein, 30 aa, Artificial Sequence
  rfr_ref_minprep_ren_neg_num_28_0002.pdb NCAP
TMRTNEILQEYKNGRHNFEGIDLANANLQN

SEQ ID NO: 93 - protein, 30 aa, Artificial Sequence
  rfr_ref_minprep_ren_neg_num_29_0005.pdb NCAP
SMHASEILQEYDNGRHDFRGIKLEDADLSG

SEQ ID NO: 94 - protein, 30 aa, Artificial Sequence
  rfr_ref_minprep_ren_neg_num_30_0005.pdb NCAP
TMRTKDILKEYNKGRHDFSGINLRNANLRN

SEQ ID NO: 95 - protein, 30 aa, Artificial Sequence
  rfr_ref_minprep_ren_neg_num_31_0005.pdb NCAP
HMQTNQILEEYNRGRHNFAGIDLQGADLRN

SEQ ID NO: 96 - protein, 30 aa, Artificial Sequence
  rfr_ref_minprep_ren_neg_num_32_0001.pdb NCAP
TMSTNEILNEYKKGRHDFSGINLKDADLSN

SEQ ID NO: 97 - protein, 30 aa, Artificial Sequence
  rfr_ref_minprep_ren_neg_num_33_0004.pdb NCAP
SMTTDKILEEYNKGRTDFRDIDLQNANLQN

SEQ ID NO: 98 - protein, 30 aa, Artificial Sequence
  rfr_ref_minprep_ren_neg_num_34_0001.pdb NCAP
SMHASKILQEYNNGRHDFANIDLAKANLEN

SEQ ID NO: 99 - protein, 30 aa, Artificial Sequence
  rfr_ref_minprep_ren_neg_num_35_0005.pdb NCAP
SMQTEQILQEYNRGRTDFAKIDLENANLKN

SEQ ID NO: 100 - protein, 30 aa, Artificial Sequence
  rfr_ref_minprep_ren_neg_num_36_0005.pdb NCAP
TMATDKILQQYKDGQHDFSGIDLANADLSK

SEQ ID NO: 101 - protein, 30 aa, Artificial Sequence
  rfr_ref_minprep_ren_neg_num_37_0002.pdb NCAP
SMQTNQILKEYNKGRHNFSGIDLQNADLSG

SEQ ID NO: 102 - protein, 30 aa, Artificial Sequence
  rfr_ref_minprep_ren_neg_num_38_0005.pdb NCAP
TMGTNEILQQYKNGQHDFADIDLKNANLQK

SEQ ID NO: 103 - protein, 30 aa, Artificial Sequence
  rfr_ref_minprep_ren_neg_num_39_0003.pdb NCAP
SMSANAILEAYDRGQRDFSKINLANANLSK

SEQ ID NO: 104 - protein, 46 aa, Artificial Sequence
  rfr_ref_minprep_ren_neg_num_20_0004.pdb CCAP
AKTKGANLRKANLEGAKLDPVLWRTANLKGARMSKKQAQEYQRANG

SEQ ID NO: 105 - protein, 46 aa, Artificial Sequence; identical to SEQ ID NO: 104
  rfr_ref_minprep_ren_neg_num_21_0004.pdb CCAP

SEQ ID NO: 106 - protein, 46 aa, Artificial Sequence
  rfr_ref_minprep_ren_neg_num_21_0003.pdb CCAP
ADTRGANLDDAKLEGAELRPVLWRTASLSGARMSKKQKQQYQRANG

SEQ ID NO: 107 - protein, 46 aa, Artificial Sequence
  rfr_ref_minprep_ren_neg_num_22_0001.pdb CCAP
AKTTGANLKRANLKGATLDPVLWRTANLEGAKMKKEQKKEYKRARG

SEQ ID NO: 108 - protein, 46 aa, Artificial Sequence
  rfr_ref_minprep_ren_neg_num_23_0004.pdb CCAP
AKTTGAELRNADLRGAKLDPVLWRTAKLTGAQMTKKQKKEYQRARG

SEQ ID NO: 109 - protein, 46 aa, Artificial Sequence
  rfr_ref_minprep_ren_neg_num_24_0002.pdb CCAP
AKTKGADLARADLRGAKLRPVLWNTARLEGAQMTKEQKKEYQRANG

SEQ ID NO: 110 - protein, 46 aa, Artificial Sequence
  rfr_ref_minprep_ren_neg_num_25_0003.pdb CCAP
AETTGAKLARADLRGAKLRPVLWNTATLTGAQMTTKQKQQYKRANG

SEQ ID NO: 111 - protein, 46 aa, Artificial Sequence
  rfr_ref_minprep_ren_neg_num_26_0004.pdb CCAP
AKTKGAKLSGADLRGAKLDPVLWNTAKLQGAKMTDNQRNEYKRANG

SEQ ID NO: 112 - protein, 46 aa, Artificial Sequence
  rfr_ref_minprep_ren_neg_num_27_0004.pdb CCAP
ANTQGAKLDNADLRGAKLRPVLWNTASLQGAKMQKKQKEQYKRAKG

SEQ ID NO: 113 - protein, 46 aa, Artificial Sequence
  rfr_ref_minprep_ren_neg_num_28_0002.pdb CCAP
AETEGADLRRADLRGATLDPVLWNKADLKGAQMKDNQRKEYKRANG

SEQ ID NO: 114 - protein, 46 aa, Artificial Sequence
  rfr_ref_minprep_ren_neg_num_29_0005.pdb CCAP
ANTQDANLQNADLRGATLDPVLWNTANLNGAQMTDKQKQEYQRANG

SEQ ID NO: 115 - protein, 46 aa, Artificial Sequence
  rfr_ref_minprep_ren_neg_num_30_0005.pdb CCAP
AETTGAKLDNADLRGAKLDPVLWNTASLSGAQMTTAQAEQYERANG

SEQ ID NO: 116 - protein, 46 aa, Artificial Sequence
  rfr_ref_minprep_ren_neg_num_31_0005.pdb CCAP
AKTTGADLANADLRGATLDPVLWRTARLTGAQMKTEQKNQYKRANG

SEQ ID NO: 117 - protein, 46 aa, Artificial Sequence
  rfr_ref_minprep_ren_neg_num_32_0001.pdb CCAP
ADTRGADLRNANLRGATLDPVLWNTADLTGAQMEAEQKKEYNRARG

SEQ ID NO: 118 - protein, 46 aa, Artificial Sequence
  rfr_ref_minprep_ren_neg_num_33_0004.pdb CCAP
ANTSGADLRNADLRGATLDPVLWNTANLKGAKMEDNQKAEYERANG

SEQ ID NO: 119 - protein, 46 aa, Artificial Sequence
  rfr_ref_minprep_ren_neg_num_34_0001.pdb CCAP
ANTSGADLENADLRGAELQPVLWRTARLQGAQMETAQKEEYKRANG

SEQ ID NO: 120 - protein, 46 aa, Artificial Sequence
  rfr_ref_minprep_ren_neg_num_35_0005.pdb CCAP
ANTKGANLDNADLRGATLDPVLWRTASLQGAKMTTRQAEEYDRARG

SEQ ID NO: 121 - protein, 46 aa, Artificial Sequence
  rfr_ref_minprep_ren_neg_num_36_0005.pdb CCAP
AETTGANLNNADLRGATLDPVLWNTASLEGAQMKKEQKKEYKRANG

SEQ ID NO: 122 - protein, 46 aa, Artificial Sequence
  rfr_ref_minprep_ren_neg_num_37_0002.pdb CCAP
ANTQGANLDNADLRGATLDPVLWNTASLEGAQMTTEEAKEYQRANG

SEQ ID NO: 123 - protein, 46 aa, Artificial Sequence
  rfr_ref_minprep_ren_neg_num_38_0005.pdb CCAP
AETEGAELNDADLRGAELAPVLWNTASLEGAKMEEKQEQQYDRARG

SEQ ID NO: 124 - protein, 46 aa, Artificial Sequence
  rfr_ref_minprep_ren_neg_num_39_0003.pdb CCAP
AETTGADLNNADLRGATLDPVLWNTAKLQGAQMTTNQKAEYQRANG

SEQ ID NO: 125 - protein, 46 aa, Artificial Sequence
  rfr_ref_minprep_ren_neg_num_40_0004.pdb CCAP
ANTRGARLQDADLRGAKLRPVLWNTANLEGAQMQTNQKAEYQRANG

SEQ ID NO: 126 - protein, 5 aa, Artificial Sequence
  rfr_ref_minprep_ren_neg_num_20_0004.pdb TAIL
KQTEG

SEQ ID NO: 127 - protein, 5 aa, Artificial Sequence
  rfr_ref_minprep_ren_neg_num_21_0003.pdb TAIL
KQTKG

SEQ ID NO: 128 - protein, 5 aa, Artificial Sequence
  rfr_ref_minprep_ren_neg_num_22_0001.pdb TAIL
QQTNG

SEQ ID NO: 129 - protein, 5 aa, Artificial Sequence
  rfr_ref_minprep_ren_neg_num_23_0004.pdb TAIL
KTTEG

SEQ ID NO: 130 - protein, 5 aa, Artificial Sequence
  rfr_ref_minprep_ren_neg_num_24_0002.pdb TAIL
QQDNG

SEQ ID NO: 131 - protein, 5 aa, Artificial Sequence
  rfr_ref_minprep_ren_neg_num_25_0003.pdb TAIL
QQDEG

SEQ ID NO: 132 - protein, 5 aa, Artificial Sequence
  rfr_ref_minprep_ren_neg_num_26_0004.pdb TAIL
QKDNG

SEQ ID NO: 133 - protein, 5 aa, Artificial Sequence
  rfr_ref_minprep_ren_neg_num_27_0004.pdb TAIL
KQDNG

SEQ ID NO: 134 - protein, 5 aa, Artificial Sequence
  rfr_ref_minprep_ren_neg_num_28_0002.pdb TAIL
QEDKG

SEQ ID NO: 135 - protein, 5 aa, Artificial Sequence
  rfr_ref_minprep_ren_neg_num_29_0005.pdb TAIL
RKTNG

SEQ ID NO: 136 - protein, 5 aa, Artificial Sequence
  rfr_ref_minprep_ren_neg_num_30_0005.pdb TAIL
KSTDG

SEQ ID NO: 137 - protein, 5 aa, Artificial Sequence
  rfr_ref_minprep_ren_neg_num_31_0005.pdb TAIL
QKDNG

SEQ ID NO: 138 - protein, 5 aa, Artificial Sequence
  rfr_ref_minprep_ren_neg_num_32_0001.pdb TAIL
QETRG

SEQ ID NO: 139 - protein, 5 aa, Artificial Sequence
  rfr_ref_minprep_ren_neg_num_33_0004.pdb TAIL
QQDKG

SEQ ID NO: 140 - protein, 5 aa, Artificial Sequence
  rfr_ref_minprep_ren_neg_num_34_0001.pdb TAIL
QSDDG

SEQ ID NO: 141 - protein, 5 aa, Artificial Sequence
  rfr_ref_minprep_ren_neg_num_35_0005.pdb TAIL
QEDKG

SEQ ID NO: 142 - protein, 5 aa, Artificial Sequence
  rfr_ref_minprep_ren_neg_num_36_0005.pdb TAIL
QSDDG

SEQ ID NO: 143 - protein, 5 aa, Artificial Sequence
  rfr_ref_minprep_ren_neg_num_37_0002.pdb TAIL
KEDRG

SEQ ID NO: 144 - protein, 5 aa, Artificial Sequence
  rfr_ref_minprep_ren_neg_num_38_0005.pdb TAIL
QSDDG

SEQ ID NO: 145 - protein, 5 aa, Artificial Sequence
  rfr_ref_minprep_ren_neg_num_39_0003.pdb TAIL
QSDDG

SEQ ID NO: 146 - protein, 5 aa, Artificial Sequence
  rfr_ref_minprep_ren_neg_num_40_0004.pdb TAIL
QQTNG

SEQ ID NO: 147 - protein, 5 aa, Artificial Sequence
  Beta solenoid domain consensus sequence
  VARIANT join(2,4..5): Wherein Xaa is any amino acid
  VARIANT 3: Wherein Xaa is Leu or Phe
AXXXX

SEQ ID NO: 148 - protein, 5 aa, Artificial Sequence
  Beta solenoid domain consensus sequence
  VARIANT 2: Wherein Xaa is Ala, Cys, Asp, Glu, Ile, Lys, Leu, Met, Asn, Arg, Ser, Thr or Val
  VARIANT 3: Wherein Xaa is Leu or Phe
  VARIANT 4: Wherein Xaa is Ala, Cys, Asp, Glu, Phe, Gly, His, Ile, Lys, Gln, Arg, Ser, Thr, Val, Trp or Tyr
  VARIANT 5: Wherein Xaa is Ala, Cys, Asp, Glu, Gly, His, Ile, Lys, Asn, Gln, Arg, Ser or Trp
AXXXX

SEQ ID NO: 149 - protein, 5 aa, Artificial Sequence
  Beta solenoid domain consensus sequence
  VARIANT join(2,4..5): Wherein Xaa is any amino acid
AXLXX

SEQ ID NO: 150 - protein, 5 aa, Artificial Sequence
  Beta solenoid domain consensus sequence
  VARIANT 2: Wherein Xaa is Ala, Cys, Asp, Glu, Ile, Lys, Leu, Met, Asn, Arg, Ser, Thr or Val
  VARIANT 4: Wherein Xaa is Ala, Cys, Asp, Glu, Phe, Gly, His, Ile, Lys, Gln, Arg, Ser, Thr, Val, Trp or Tyr
  VARIANT 5: Wherein Xaa is Ala, Cys, Asp, Glu, Gly, His, Ile, Lys, Asn, Gln, Arg, Ser or Trp
AXLXX

SEQ ID NO: 151 - protein, 5 aa, Artificial Sequence
  Beta solenoid domain consensus sequence
  VARIANT 2: Wherein Xaa is Asp or Asn
  VARIANT 4: Wherein Xaa is Cys, Arg, His, Lys, Asp, Glu, Ser, Thr, Asn or Gln
  VARIANT 5: Wherein Xaa is any amino acid
AXLXX

SEQ ID NO: 152 - protein, 7 aa, Artificial Sequence
  Beta solenoid domain consensus sequence
  VARIANT 1: Wherein Xaa is Ala, Gly, Ser or Thr
  VARIANT join(2,4,6..7): Wherein Xaa is any amino acid
  VARIANT 3: Wherein Xaa is Ala, Gly or Val
  VARIANT 5: Wherein Xaa is Ala or Gly
XXXXXXX

SEQ ID NO: 153 - protein, 14 aa, Artificial Sequence
  Beta solenoid domain consensus sequence
  VARIANT 1,8: Wherein Xaa is Ser, Gly, Thr or Ala
  VARIANT join(2,4,6..7,13..14): Wherein Xaa is any amino acid
  VARIANT 3,10: Wherein Xaa is Ala, Val or Gly
  VARIANT 5,12: Wherein Xaa is Ala or Gly
  VARIANT 9,11: Wherein Xaa is Gly, Ala, Val, Leu, Ile, Pro, Phe, Met or Trp
XXXXXXXXXXXXXX

SEQ ID NO: 154 - protein, 14 aa, Artificial Sequence
  Beta solenoid domain consensus sequence
  VARIANT join(2,4,6..7,13..14): Wherein Xaa is any amino acid
  VARIANT 9,11: Wherein Xaa is Gly, Ala, Val, Leu, Ile, Pro, Phe, Met or Trp
SXAXGXXSXAXGXX

SEQ ID NO: 155 - protein, 15 aa, Artificial Sequence
  Beta solenoid domain consensus sequence
  VARIANT join(2,4,6..7,14..15): Wherein Xaa is any amino acid
  VARIANT 10: Wherein Xaa is Ile or Val
  VARIANT 11: Wherein Xaa is Gly or Ala
NXAXGXXSTXXGGXX

SEQ ID NO: 156 - protein, 15 aa, Artificial Sequence
  Beta solenoid domain consensus sequence
  VARIANT join(2,4,6..7,14..15): Wherein Xaa is any amino acid
NXAXGXXSTIGGGXX

SEQ ID NO: 157 - protein, 19 aa, Artificial Sequence
  Beta solenoid domain consensus sequence
  VARIANT join(2,4,6..7,10,12..13,15,17,18): Wherein Xaa is any amino aicd
  VARIANT 5,16: Wherein Xaa is Val, Ile or Leu
GXQXXXXGGXAXXTXXXXG

SEQ ID NO: 158 - protein, 880 aa, Artificial Sequence
  SynRFR24.nnum35.x4
MGSSHHHHHHSSGLVPRGSSMQTEQILQEYNRGRTDFAKIDLENANLKNAELAGADLANANLHRANLENANLANAKLEEANLEEANLAGADLRNANLQRANLARADLAGADLTGANLAEADLREARLQKANLENADLTNADLTGADLEGARLHGANLEGANLTNANLRKANLENADLRNADLTGANTKGANLDNADLRGATLDPVLWRTASLQGAKMTTRQAEEYDRARGGGGSSMQTEQILQEYNRGRTDFAKIDLENANLKNAELAGADLANANLHRANLENANLANAKLEEANLEEANLAGADLRNANLQRANLARADLAGADLTGANLAEADLREARLQKANLENADLTNADLTGADLEGARLHGANLEGANLTNANLRKANLENADLRNADLTGANTKGANLDNADLRGATLDPVLWRTASLQGAKMTTRQAEEYDRARGGGGSSMQTEQILQEYNRGRTDFAKIDLENANLKNAELAGADLANANLHRANLENANLANAKLEEANLEEANLAGADLRNANLQRANLARADLAGADLTGANLAEADLREARLQKANLENADLTNADLTGADLEGARLHGANLEGANLTNANLRKANLENADLRNADLTGANTKGANLDNADLRGATLDPVLWRTASLQGAKMTTRQAEEYDRARGGGGSSMQTEQILQEYNRGRTDFAKIDLENANLKNAELAGADLANANLHRANLENANLANAKLEEANLEEANLAGADLRNANLQRANLARADLAGADLTGANLAEADLREARLQKANLENADLTNADLTGADLEGARLHGANLEGANLTNANLRKANLENADLRNADLTGANTKGANLDNADLRGATLDPVLWRTASLQGAKMTTRQAEEYDRARGQEDKG

SEQ ID NO: 159 - protein, 880 aa, Artificial Sequence
  SynRFR24.nnum36.x4
MGSSHHHHHHSSGLVPRGSTMATDKILQQYKDGQHDFSGIDLANADLSKAELAGADLSGADLTRADLRDANLANADLQEANLAEAKLQGANLENANLARADLSRANLAGADLHGANLAEADLRNADLRNANLQNADLRKARLQGADLEGANLEGANLHGADLENADLARADLQKADLRNANLTGAETTGANLNNADLRGATLDPVLWNTASLEGAQMKKEQKKEYKRANGGGGSTMATDKILQQYKDGQHDFSGIDLANADLSKAELAGADLSGADLTRADLRDANLANADLQEANLAEAKLQGANLENANLARADLSRANLAGADLHGANLAEADLRNADLRNANLQNADLRKARLQGADLEGANLEGANLHGADLENADLARADLQKADLRNANLTGAETTGANLNNADLRGATLDPVLWNTASLEGAQMKKEQKKEYKRANGGGGSTMATDKILQQYKDGQHDFSGIDLANADLSKAELAGADLSGADLTRADLRDANLANADLQEANLAEAKLQGANLENANLARADLSRANLAGADLHGANLAEADLRNADLRNANLQNADLRKARLQGADLEGANLEGANLHGADLENADLARADLQKADLRNANLTGAETTGANLNNADLRGATLDPVLWNTASLEGAQMKKEQKKEYKRANGGGGSTMATDKILQQYKDGQHDFSGIDLANADLSKAELAGADLSGADLTRADLRDANLANADLQEANLAEAKLQGANLENANLARADLSRANLAGADLHGANLAEADLRNADLRNANLQNADLRKARLQGADLEGANLEGANLHGADLENADLARADLQKADLRNANLTGAETTGANLNNADLRGATLDPVLWNTASLEGAQMKKEQKKEYKRANGQSDDG

SEQ ID NO: 160 - protein, 880 aa, Artificial Sequence
  SynRFR24.nnum40.x4
MGSSHHHHHHSSGLVPRGSSMHEDEILDEYNNGRKNFSGIDLQGADLEDAELAGADLSDANLEQANLQNANLANANLENANLQDADLHGARLQNADLRGANLEDADLANARLEGANLAEADLRRADLRGADLTNADLEDADLEGANLHGARLEGANLRGANLTDARLENADLSGADLRNANLEGANTRGARLQDADLRGAKLRPVLWNTANLEGAQMQTNQKAEYQRANGGGGSSMHEDEILDEYNNGRKNFSGIDLQGADLEDAELAGADLSDANLEQANLQNANLANANLENANLQDADLHGARLQNADLRGANLEDADLANARLEGANLAEADLRRADLRGADLTNADLEDADLEGANLHGARLEGANLRGANLTDARLENADLSGADLRNANLEGANTRGARLQDADLRGAKLRPVLWNTANLEGAQMQTNQKAEYQRANGGGGSSMHEDEILDEYNNGRKNFSGIDLQGADLEDAELAGADLSDANLEQANLQNANLANANLENANLQDADLHGARLQNADLRGANLEDADLANARLEGANLAEADLRRADLRGADLTNADLEDADLEGANLHGARLEGANLRGANLTDARLENADLSGADLRNANLEGANTRGARLQDADLRGAKLRPVLWNTANLEGAQMQTNQKAEYQRANGGGGSSMHEDEILDEYNNGRKNFSGIDLQGADLEDAELAGADLSDANLEQANLQNANLANANLENANLQDADLHGARLQNADLRGANLEDADLANARLEGANLAEADLRRADLRGADLTNADLEDADLEGANLHGARLEGANLRGANLTDARLENADLSGADLRNANLEGANTRGARLQDADLRGAKLRPVLWNTANLEGAQMQTNQKAEYQRANGQQTNG

SEQ ID NO: 161 - protein, 910 aa, Artificial Sequence
  SynRFR24.nnum35.nc.ll.x4.K129S
MGSSHHHHHHSSGLVPRGSRMRRDEILEEYRRGRRNFQHINLQEIELTNAELAGADLANANLHRANLENANLANAKLEEANLEEANLAGADLRNANLQRANLARADLAGADLTGANLAEADLREARLQSANLENADLTNADLTGADLEGARLHGANLEGANLTNANLRKANLENADLRNADLTGARTTGARLDDADLRGATVDPVLWRTASLRGAKMEEEQRREYERARGGGGSAAAAAAGGGSRMRRDEILEEYRRGRRNFQHINLQEIELTNAELAGADLANANLHRANLENANLANAKLEEANLEEANLAGADLRNANLQRANLARADLAGADLTGANLAEADLREARLQKANLENADLTNADLTGADLEGARLHGANLEGANLTNANLRKANLENADLRNADLTGARTTGARLDDADLRGATVDPVLWRTASLRGAKMEEEQRREYERARGGGGSAAAAAAGGGSRMRRDEILEEYRRGRRNFQHINLQEIELTNAELAGADLANANLHRANLENANLANAKLEEANLEEANLAGADLRNANLQRANLARADLAGADLTGANLAEADLREARLQKANLENADLTNADLTGADLEGARLHGANLEGANLTNANLRKANLENADLRNADLTGARTTGARLDDADLRGATVDPVLWRTASLRGAKMEEEQRREYERARGGGGSAAAAAAGGGSRMRRDEILEEYRRGRRNFQHINLQEIELTNAELAGADLANANLHRANLENANLANAKLEEANLEEANLAGADLRNANLQRANLARADLAGADLTGANLAEADLREARLQKANLENADLTNADLTGADLEGARLHGANLEGANLTNANLRKANLENADLRNADLTGARTTGARLDDADLRGATVDPVLWRTASLRGAKMEEEQRREYERARGQEDKG

SEQ ID NO: 162 - protein, 880 aa, Artificial Sequence
  SynRFR24.nnum36.nc.x4
MGSSHHHHHHSSGLVPRGSRMRRDEILEEYRRGRRNFQHINLQEIELTNAELAGADLSGADLTRADLRDANLANADLQEANLAEAKLQGANLENANLARADLSRANLAGADLHGANLAEADLRNADLRNANLQNADLRKARLQGADLEGANLEGANLHGADLENADLARADLQKADLRNANLTGARTTGARLDDADLRGATVDPVLWRTASLRGAKMEEEQRREYERARGGGGSRMRRDEILEEYRRGRRNFQHINLQEIELTNAELAGADLSGADLTRADLRDANLANADLQEANLAEAKLQGANLENANLARADLSRANLAGADLHGANLAEADLRNADLRNANLQNADLRKARLQGADLEGANLEGANLHGADLENADLARADLQKADLRNANLTGARTTGARLDDADLRGATVDPVLWRTASLRGAKMEEEQRREYERARGGGGSRMRRDEILEEYRRGRRNFQHINLQEIELTNAELAGADLSGADLTRADLRDANLANADLQEANLAEAKLQGANLENANLARADLSRANLAGADLHGANLAEADLRNADLRNANLQNADLRKARLQGADLEGANLEGANLHGADLENADLARADLQKADLRNANLTGARTTGARLDDADLRGATVDPVLWRTASLRGAKMEEEQRREYERARGGGGSRMRRDEILEEYRRGRRNFQHINLQEIELTNAELAGADLSGADLTRADLRDANLANADLQEANLAEAKLQGANLENANLARADLSRANLAGADLHGANLAEADLRNADLRNANLQNADLRKARLQGADLEGANLEGANLHGADLENADLARADLQKADLRNANLTGARTTGARLDDADLRGATVDPVLWRTASLRGAKMEEEQRREYERARGQSDDG

SEQ ID NO: 163 - DNA, 2643 bp, Artificial Sequence
  SynRFR24.nnum36.nc.x4
atgggtagcagccatcaccatcatcatcatagcagcggtctggttccgcgtggtagccgtatgcgtcgtgatgaaattctggaagaatatcgtcgtggtcgtcgtaactttcagcatattaatctgcaagaaatcgaactgaccaatgcagaactggcaggcgcagatctgagcggtgccgatctgacccgtgcggatctgcgtgatgcaaatctggcaaacgcagacctgcaagaagccaatctggccgaagcaaaactgcagggtgcgaatctggaaaatgccaacctggctcgtgctgatctgtcacgtgctaatttagccggtgccgacctgcatggtgcaaacctggcggaagccgatctgcgcaatgcggatttacgtaatgccaatctgcagaatgcggacctgcgtaaagcacgtctgcaaggggcagatctggaaggtgctaacctggaaggcgcaaatttacatggtgcagatttagaaaacgccgatctggctcgcgcagatttacagaaagctgatctgcgtaacgcgaatctgaccggtgcacgtaccaccggtgcgcgtctggatgatgccgatttacgcggtgcaaccgttgatccggttctgtggcgtaccgcaagcctgcgtggtgccaaaatggaagaagaacagcgtcgcgaatatgaacgtgcccgtggtggtggcggttctcgcatgcgtagagatgaaatcttagaagagtaccgtcgcggacgtcgcaattttcaacatatcaacttacaagagatcgagctgacaaacgccgaattagcgggtgctgatttaagcggagcggatttaacacgtgcagacttacgtgatgcgaacctggccaatgccgatcttcaagaagcaaatttagcagaggccaaattacagggtgccaaccttgaaaacgctaatcttgcgcgtgcagacctgagtcgtgctaaccttgccggtgcagatcttcacggtgccaatcttgcggaggctgacctgcggaatgcagaccttcgcaacgcgaacctgcaaaacgcggatcttcgcaaagctcgcctgcaaggtgccgacttagaaggtgcgaatttagagggtgctaatcttcatggtgcggaccttgagaacgcggatttagctagagctgatcttcagaaagccgacttacgcaatgcaaatttaacaggcgctcgcaccacaggtgcacgcttagatgacgctgatttgcgtggcgctacagttgaccctgtgctgtggcgcacagccagcttacgtggcgctaagatggaagaggaacaacgccgtgagtacgaacgtgcacgcggtggcggtggcagtcggatgcgtcgggacgagattttagaggaataccgtagaggtcgcagaaattttcagcacataaaccttcaagaaattgagcttacgaatgcggaacttgctggggctgatctgagtggggcagacttaactagagccgaccttcgtgatgccaatttagcgaacgccgatttgcaagaggcgaatttggcggaggcgaaacttcaaggtgcaaacttagagaatgcgaacttagcaagagcggatctgagtcgcgcaaatcttgctggcgcagacttgcatggtgccaatttggcagaggcagatcttcgtaacgctgatttacggaacgcaaatcttcagaacgcagatttgcggaaagcacgccttcagggtgctgatcttgagggtgcaaatttggaaggggcaaacttgcacggtgctgacttggagaacgctgacctggcacgagcggacttgcagaaagcagacctgagaaatgcaaatctgactggcgcacgcacaactggcgctcgtttagatgatgcggacttaagaggtgccacagtagatccggttttatggcgcacggcatcattacggggagcaaaaatggaagaggagcaaagacgtgaatatgagcgtgctcgcggaggtggtggctcccgcatgcgacgcgacgagatccttgaagagtatcgcagaggccgtcggaatttccaacacattaacctgcaagagatagagttaactaatgccgagcttgctggtgccgatttatctggtgcggatttgactcgagcggaccttcgggacgcaaaccttgcgaatgctgatttacaagaagctaacctggctgaggccaagctgcaaggcgctaatttggaaaatgcgaatcttgcacgggcagatttatcaagagccaaccttgctggggcagatttacatggggctaatctggctgaagctgaccttcgtaatgctgatcttagaaatgcaaacctgcagaacgctgacttacgtaaagcccgtttgcagggtgcagaccttgaaggcgctaacttagagggtgccaacttacatggcgcagatcttgagaatgcagatctggcaagagccgatctgcaaaaggccgatctgagaaacgccaacctgacaggtgctagaaccacgggtgctcgcctggacgatgcagacctgcgtggcgcaaccgtagatccagtactttggagaaccgcatctcttcgcggagccaagatggaggaggagcagcgaagagaatatgaaagagcacgcggtcagtcagatgatggttaa

SEQ ID NO: 164 - DNA, 2733 bp, Artificial Sequence
  SynRFR24.nnum35.nc.ll.x4.K129S
atgggtagcagccatcaccatcatcatcatagcagcggtctggttccgcgtggtagccgtatgcgtcgtgatgaaattctggaagaatatcgtcgtggtcgtcgtaactttcagcatattaatctgcaagaaatcgaactgaccaatgcagaactggcaggcgcagatctggcaaatgcaaatctgcatcgtgccaatctggaaaatgccaacctggccaatgcgaaactggaagaagcaaatctggaagaggccaatcttgccggtgccgatctgcgtaacgccaacctgcagcgtgcaaacctggcacgtgcggatttagcgggtgcagatctgaccggtgcgaatctggccgaagcggatctgcgtgaagcacgtctgcagagtgcgaacctggaaaacgccgatctgactaatgcggacctgacaggtgccgacctggaaggtgcccgtctgcatggtgcaaatttagaaggcgcaaatctgaccaacgccaatctgcgcaaagccaatttggagaatgcagacctgcgtaatgctgatttaaccggtgcacgtaccaccggtgcgcgtctggatgatgccgatttacgtggtgcaaccgttgatccggttctgtggcgtaccgcaagcctgcgtggtgccaaaatggaagaagaacagcgtcgcgaatatgaacgtgcccgtggtggtggcggtagcgcagctgcagcagcagccggtggtggttctcgcatgcgtagagatgaaatcttagaagagtaccgtcgcggacgtcgcaattttcaacatatcaacttacaagagatcgagctgacaaacgccgaattagctggcgcagatttagcgaatgccaacttacatcgtgcgaacttagaaaatgctaatctggcgaacgccaaattagaagaagctaacttagaagaggcgaaccttgcgggtgctgatttacgtaatgcgaatctgcaacgcgcaaatcttgctcgtgcggatcttgcaggggctgatcttacaggtgctaacctggcggaagcagacttacgcgaggctcgtttacagaaagctaatcttgagaatgctgatctgacaaatgccgatcttaccggtgcagacttagaaggtgcacgcttacatggcgcaaaccttgaaggtgcgaacctgacgaacgcaaatttaagaaaagcgaatttagaaaatgcggacctgcgcaacgcagacctgacgggtgcgcgtaccacaggcgcacgcttagatgatgcagatcttcgcggtgccacagtggaccctgtgctgtggcgcacagcctcactgagaggcgctaagatggaagaggaacaacgccgtgagtacgaacgtgcacgcggtggcggtggttcagcagcagctgccgcagcaggtggaggttcacgtatgcgacgcgacgaaattttagaggaatatagacgcggtcgccgtaatttccagcacatcaaccttcaagaaattgagttaacaaatgcggagttagccggtgcggacctggccaacgctaatcttcaccgtgctaatttagagaacgcgaatttagctaacgccaaacttgaggaagccaatcttgaagaagcaaacttggctggtgcggacttacgcaacgcaaacttacaacgagccaatttagcacgtgccgaccttgctggtgcagaccttacaggggcaaatttggcggaggctgatctgcgcgaggcaagactgcaaaaagcaaacttagagaatgccgacttaaccaatgcggatttaacaggggcagaccttgaaggcgcacgcctgcacggtgccaacttagagggtgccaaccttacaaacgcgaatcttcgtaaagcgaaccttgagaacgcggatttacgcaatgccgatctgacaggcgcacgtacaacaggtgcacgcctggacgacgccgacctgcgtggcgctacagttgatcctgtgttatggcgtacagcgagcttacgcggagcaaaaatggaagaggagcaaagacgtgaatatgagcgtgctcgcggaggtggtggctctgcagccgcagcagcggcaggcggtggaagtagaatgcgtcgggacgaaatccttgaggaataccgacgtggcagacggaactttcaacacataaacctgcaagagatagaacttacgaacgcggagcttgcaggcgcagaccttgcgaacgctaaccttcatagagcaaacttggaaaacgcgaacttagccaatgcaaaattagaagaggcaaatttagaagaagccaacctggccggcgcagatcttcgtaatgctaatttacagcgtgccaatcttgcacgcgctgacttagccggtgcagatttaactggggcaaatcttgccgaagcagatttaagagaagctcgccttcagaaagccaacttagaaaacgcagatttaaccaacgcagatcttactggcgctgatttggagggtgctagattacacggtgcaaacctggaaggcgcaaaccttactaatgctaacctgcgtaaggctaatctggaaaacgctgacctgcgtaacgcggatcttacgggtgctcgcaccacgggtgccagactggatgacgctgatcttcggggagcgacagtagatccagttctttggcgcacggccagtttacggggtgcaaagatggaggaagagcagcgaagagaatatgaaagagcacgcggtcaagaagataaaggctaa

SEQ ID NO: 165 - DNA, 2643 bp, Artificial Sequence
  SynRFR24.nnum35.x4
atgggcagcagccatcaccatcatcatcatagcagcggtctggttccgcgtggtagcagcatgcagaccgagcagattctgcaagaatataatcgtggtcgtaccgatttcgccaaaattgatctggaaaatgccaatctgaaaaacgcagaactggcaggcgcagatctggccaatgcaaatctgcatcgtgcaaacctggaaaacgcgaacctggcgaatgccaaactggaagaagcgaatctggaagaggccaaccttgccggtgccgatctgcgtaatgccaacctgcagcgtgctaatctggcacgtgcggatttagcgggtgcagatctgaccggtgctaacctggccgaagcggatctgcgtgaagcacgtctgcagaaagcaaatttagaaaatgcggatctgaccaacgccgatttaaccggtgcggacctggaaggtgcccgtctgcatggtgccaatttagaaggcgcaaatctgacaaatgcgaacctgcgtaaggcaaatcttgaaaacgctgatttacgtaacgccgatctgactggcgcaaataccaaaggtgccaatcttgataatgcagacctgcgtggtgcaaccttagatccggttctgtggcgtaccgcaagcctgcagggtgcaaaaatgaccacacgtcaggccgaagaatatgaccgtgcacgcggtggtggtggttcaagtatgcagacagaacaaatccttcaagagtacaatcgcggtcgcacagactttgcaaaaattgatttagagaacgccaacctgaagaatgcagaattagctggtgccgacctggctaacgcgaatttacatagagccaacttagagaatgcgaatcttgcaaatgccaaattagaggaagcaaacttagaagaggcaaatcttgctggtgcagatttacgtaatgcaaatttacagcgtgcaaatttagcccgtgctgatcttgcgggtgctgacttaacaggggcaaatctggcggaagccgatttacgcgaggctcgtttacagaaagcgaaccttgagaacgcggacctgacaaacgcggatcttacaggtgcagacttagaaggtgcacgcttacatggcgctaatcttgaaggtgcgaaccttaccaacgccaatctgcgcaaggcgaacttggagaatgctgatctgcgcaatgctgacctgacaggtgccaacacaaagggtgcgaacttagataacgcagatcttcgcggtgccacactggaccctgtgctgtggcgcacagcctcattacagggtgccaagatgacaactcgccaagcagaagaatacgatcgcgcacgtggcggtggcggtagctcaatgcaaaccgaacaaattttacaagagtataacagaggccgtaccgactttgcgaagatcgaccttgaaaatgctaaccttaaaaatgccgagttagctggcgctgacttagcaaacgctaacttacatcgagctaatttggagaacgctaatttagccaacgcgaaacttgaggaagctaaccttgaagaggcgaacctggctggcgcagacctgcgcaatgccaatcttcaacgtgcgaatttagctcgcgcagatttagcaggggctgaccttacgggtgcgaatctggctgaggccgatcttcgtgaggcaagactgcaaaaagctaatctggaaaacgccgacctgaccaatgcggacttgactggggcagaccttgaaggcgctcgcctgcatggcgcaaacttggagggtgctaatttgactaacgcaaacttacgcaaagccaacttggaaaacgcagacttgcgtaatgcggatttgacaggtgcgaatacgaaaggcgctaacctggataatgccgacttacgcggtgctacccttgatccggtgttatggcgcaccgcgtcacttcaaggggctaaaatgacaaccagacaggcggaagagtacgatagagcccgtggtggcggaggttcatctatgcaaactgagcagatcttacaagaatacaaccgaggacgcacggattttgctaaaatcgatcttgagaacgcaaatcttaagaatgccgaacttgccggtgctgatttagctaatgctaatcttcatagagccaaccttgaaaacgccaatctggccaacgcaaaattagaagaagccaacctggaagaggctaatcttgcaggggctgatctgcggaacgcgaatctgcaacgcgcaaacttagcgcgtgccgacttagctggtgcggatttaactggtgccaaccttgcggaagccgacctgcgcgaggcacgccttcaaaaagcgaacctggaaaatgcggatttaaccaatgcagatctgacaggggctgatttggaaggcgcaagactgcatggtgcgaatcttgagggtgcaaacttgaccaatgcaaacctgcgcaaagctaaccttgagaatgcagatcttcgtaatgccgatttaacgggtgcaaacacaaaaggtgcaaatctggacaacgcggatcttcgtggtgcgacattagatcctgttttatggcggacagcatctctgcaaggtgcgaagatgacgacccgtcaagcggaagagtacgaccgtgcacgtggtcaagaagataaaggttaa

SEQ ID NO: 166 - DNA, 2643 bp, Artificial Sequence
  SynRFR24.nnum36.x4
atgggcagcagccatcaccatcatcatcatagcagcggtctggttccgcgtggtagcaccatggcaaccgataaaattctgcagcagtataaagatggccagcatgattttagcggtattgatctggcaaatgcagatctgagcaaagccgaactggcaggcgcagatctgtcaggtgccgatctgacccgtgcggatctgcgtgatgcaaatctggccaacgccgatctgcaagaagccaatctggccgaagcaaaactgcagggtgcgaatctggaaaatgctaatctggcacgtgctgatctgtctcgtgcaaatttagccggtgcagacctgcatggtgcaaacctggcggaagctgatctgcgtaacgccgacctgcgcaatgccaatctgcagaatgcggacctgcgtaaagcacgtctgcaaggggcagatctggaaggtgctaacctggaaggcgcaaatttacatggtgccgatttagaaaacgcagatttagcgcgtgcagatttacagaaagccgatttacgtaacgcaaatctgaccggtgccgaaaccaccggtgccaacctgaataatgcggatttacgtggtgcaaccttagatccggttctgtggaataccgcaagcttagaaggtgcacagatgaaaaaagagcagaaaaaagaatacaagcgtgccaatggtggtggtggcagtaccatggccacagataagatccttcaacaatataaagacggtcagcacgacttttcaggcatcgatctggcgaacgcggatttaagtaaagcagaacttgcgggtgccgacctgagcggagcagatttaacacgtgccgacttacgtgatgcgaacttagcaaacgctgacctgcaagaggcgaatttagcagaggccaaattacagggtgctaacttagaaaatgccaatttagcaagagcggatctgagtcgtgccaaccttgctggtgcagatcttcacggtgctaatcttgccgaggccgatcttcgcaatgcggatcttcggaacgcaaacctgcaaaatgcagacttaagaaaagctcgcctgcaaggtgcggacttagagggtgcaaatcttgaaggggcaaaccttcatggcgcagacctggaaaacgcggacctggcacgggcagaccttcagaaagcagacttacgcaatgcgaatttaacaggtgcagaaacaactggcgctaatctgaacaatgccgaccttcgcggtgcaacactggaccctgtgctgtggaacacagcctcacttgagggtgcccaaatgaagaaagaacaaaagaaagaatataaacgcgcaaatggcggtggcggttcaacaatggcgacggacaaaatcctgcaacagtacaaggacggacaacatgatttctctggtatcgacctggctaacgctgatctttcaaaagcagaattagctggggctgatctgagtggtgcggatttaactagagccgatctgcgcgacgccaacctggctaatgccgacttgcaagaggctaacctggcagaggcgaaactgcaaggcgctaaccttgagaatgcgaatcttgctagagcagacctgtcacgcgcaaaccttgccggtgctgatttacatggcgctaacttggccgaggcagacctgagaaacgcagatcttcgtaatgcaaatcttcagaatgcagatcttcgcaaagcgcgtctgcagggtgccgaccttgaaggtgcaaatttagaaggtgcgaacttacatggtgctgatcttgagaatgccgatttagcccgtgccgatcttcaaaaagctgacctgcggaatgcgaacctgacaggtgcggaaacgacaggtgcaaacttaaacaacgcggacttacgcggtgccacgcttgacccggtgttatggaatacagccagccttgaaggcgctcaaatgaaaaaagagcaaaaaaaagaatataaacgagccaacggtggcggtggctctacgatggctactgataaaatcttgcagcaatacaaggatgggcagcacgatttcagtggcattgatttagctaacgcagacttgtctaaagccgagttagctggtgcggacctttctggcgctgacttaactcgagctgaccttcgtgacgccaatcttgcaaacgctgatttacaagaagcaaatcttgcggaagccaaattacaaggcgcaaatctggaaaacgcaaacttagctcgcgcagacttatcaagagctaatttagctggcgcagatttacacggtgcgaacctggccgaagcagatttacgtaatgcagacctgcgcaacgcaaaccttcagaacgctgatttgcgtaaagcccgtttacagggtgctgatttggaaggtgccaatcttgagggtgctaatctgcatggggcagacttagagaatgcggatttggcacgtgcggacttgcagaaagcggatttgagaaatgctaacttaaccggtgcggagacaaccggtgcgaatcttaataatgccgatcttagaggtgcgacccttgatccagttttatggaacaccgcatcattagagggtgcccagatgaaaaaagagcaaaagaaagaatacaaacgtgcgaacggtcagtcagatgatggttaa

SEQ ID NO: 167 - DNA, 2643 bp, Artificial Sequence
  SynRFR24.nnum40.x4
atgggcagcagccatcaccatcatcatcatagcagcggtctggttccgcgtggtagcagcatgcatgaagatgaaattctggatgagtataacaacggtcgcaaaaactttagcggtattgatctgcagggtgcagatctggaagatgcagaactggcaggcgcagatctgagtgatgcaaatctggaacaggcaaatctgcagaatgccaatctggccaatgccaacctggaaaatgcgaatctgcaggacgccgacctgcatggtgctcgtctgcagaacgcggatctgcgtggcgcaaatttagaagatgccgatctggcgaacgcacgtctggaaggcgctaatctggccgaagccgatctgcgtcgtgcagacttacgtggtgcggatctgaccaatgcggatttagaggatgcggacctggaaggtgcaaatttacatggtgcacgtttagaaggtgcgaacctgcgtggtgccaatcttaccgatgcgcgtctggaaaacgccgatctgagcggtgccgatttacgtaacgcgaatcttgaaggcgcaaatacccgtggtgcacgcctgcaagatgctgatttacgcggtgcaaaactgcgtccggttctgtggaataccgccaacttagaaggcgcacagatgcagaccaatcagaaagcagaatatcagcgtgcaaatggtggtggtggcagctcaatgcacgaggatgaaatccttgacgaatacaataatggccgtaagaatttttccggcatcgatttacagggtgccgaccttgaggatgccgaattagccggtgctgatctgtcagacgcgaatttagaacaggccaatttacagaacgcaaacctggcaaacgcaaacttagaaaacgccaaccttcaggatgctgatcttcatggcgcacgcttacagaatgcagatcttcgcggagcgaaccttgaagatgctgacctggcaaatgctcgccttgagggtgcgaatctggcagaggcagatttacgcagagcggaccttcgtggtgcagatttaacaaacgctgatcttgaggacgctgacttagagggtgcaaaccttcacggtgctagacttgaaggggctaacttacgcggagccaatctgacagacgctcgtttagaaaatgcagacctgagcggagctgatctgcgcaacgccaatctggaaggtgccaatacacgcggtgcccgtttacaggacgcggatttacggggagcgaaattacgtccggtgttatggaatacagcaaaccttgaaggtgcccaaatgcagacaaaccaaaaagccgagtatcaacgtgccaacggtggcggaggttcaagtatgcatgaggacgagattttggacgagtacaacaatggaagaaaaaacttctcaggcatcgatctgcaaggcgcagacttggaggacgcagaacttgccggtgccgacttatcagatgctaaccttgaacaagccaatcttcaaaatgctaatcttgcaaacgctaatttggagaatgcgaacttacaagatgcggatctgcacggtgctcgcttgcaaaatgccgacttgcgaggggcaaacttggaagatgcggacttagccaatgcacggttggagggtgctaatttagcggaagcagaccttcgtcgcgctgaccttcggggagccgacctgaccaacgctgacctggaagatgccgatttagaaggtgcaaatctgcatggcgctcgcctggaaggcgcaaacttgcgtggtgctaacctgacagatgcacggcttgaaaacgcggacctgtcaggggcagacctgcgtaatgccaatttggagggtgcgaacacccgtggggcacgtttacaagacgccgatcttagaggcgctaaacttcgtcctgttttatggaacaccgctaatttagagggtgcccagatgcaaacgaatcaaaaggcggaataccaacgtgcgaatggcggaggcggtagtagtatgcacgaagatgagattttggatgaatacaataacggacgcaagaacttctctggaattgacctgcaaggtgcggacttagaagatgctgagttagcgggtgccgatctgagtgacgccaaccttgagcaggccaacctgcagaacgcaaatttagcaaatgcgaatttggaaaacgctaacctgcaagacgcggacttacatggcgcaagactgcaaaatgcggatcttcggggtgctaacttagaggacgccgatttagcgaatgctcggttagaaggggcaaacctggcggaagcggatttacgtcgtgctgatctgcgtggggcagatctgacaaatgccgatcttgaagatgcagatcttgagggtgccaacttgcatggtgcacgacttgaaggtgccaatttacgtggcgcaaatctgaccgacgcacgcctggaaaatgcagatctttctggtgccgatctgcgtaatgcaaacctggaaggggctaatacgcgtggcgctcggctgcaggatgccgacttaagaggcgcaaaattacgccctgtgctgtggaacacggcgaacttggaaggtgcgcaaatgcaaactaatcagaaagctgagtaccaacgcgctaatggtcagcagacaaatggttaa

SEQ ID NO: 168 - protein, 14 aa, Artificial Sequence
  Linker sequence
GGGSAAAAAAGGGS

SEQ ID NO: 169 - protein, 135 aa, Artificial Sequence
  Solenoid domain sequence K129S
AELAGADLANANLHRANLENANLANAKLEEANLEEANLAGADLRNANLQRANLARADLAGADLTGANLAEADLREARLQSANLENADLTNADLTGADLEGARLHGANLEGANLTNANLRKANLENADLRNADLTG

SEQ ID NO: 170 - protein, 1310 aa, Artificial Sequence
  SynRFR24_nc.x6_1
MGSSHHHHHHSSGLVPRGSRMRRDEILEEYRRGRRNFQHINLQEIELTNASLTGADLSYANLHHANLSRANLRSADLRNANLSHANLSGANLEEANLEAANLRGADLHEANLSGADLQEANLTQANLKDANLSDANLEQADLAGADLQGAVLDGANLHGANLNNANLSEAMLTRANLEQADLSGARTTGARLDDADLRGATVDPVLWRTASLRGAKMEEEQRREYERARGGGGSRMRRDEILEEYRRGRRNFQHINLQEIELTNASLTGADLSYANLHHANLSRANLRSADLRNANLSHANLSGANLEEANLEAANLRGADLHEANLSGADLQEANLTQANLKDANLSDANLEQADLAGADLQGAVLDGANLHGANLNNANLSEAMLTRANLEQADLSGARTTGARLDDADLRGATVDPVLWRTASLRGAKMEEEQRREYERARGGGGSRMRRDEILEEYRRGRRNFQHINLQEIELTNASLTGADLSYANLHHANLSRANLRSADLRNANLSHANLSGANLEEANLEAANLRGADLHEANLSGADLQEANLTQANLKDANLSDANLEQADLAGADLQGAVLDGANLHGANLNNANLSEAMLTRANLEQADLSGARTTGARLDDADLRGATVDPVLWRTASLRGAKMEEEQRREYERARGGGGSRMRRDEILEEYRRGRRNFQHINLQEIELTNASLTGADLSYANLHHANLSRANLRSADLRNANLSHANLSGANLEEANLEAANLRGADLHEANLSGADLQEANLTQANLKDANLSDANLEQADLAGADLQGAVLDGANLHGANLNNANLSEAMLTRANLEQADLSGARTTGARLDDADLRGATVDPVLWRTASLRGAKMEEEQRREYERARGGGGSRMRRDEILEEYRRGRRNFQHINLQEIELTNASLTGADLSYANLHHANLSRANLRSADLRNANLSHANLSGANLEEANLEAANLRGADLHEANLSGADLQEANLTQANLKDANLSDANLEQADLAGADLQGAVLDGANLHGANLNNANLSEAMLTRANLEQADLSGARTTGARLDDADLRGATVDPVLWRTASLRGAKMEEEQRREYERARGGGGSRMRRDEILEEYRRGRRNFQHINLQEIELTNASLTGADLSYANLHHANLSRANLRSADLRNANLSHANLSGANLEEANLEAANLRGADLHEANLSGADLQEANLTQANLKDANLSDANLEQADLAGADLQGAVLDGANLHGANLNNANLSEAMLTRANLEQADLSGARTTGARLDDADLRGATVDPVLWRTASLRGAKMEEEQRREYERARGKSDDG

SEQ ID NO: 171 - DNA, 3933 bp, Artificial Sequence
  SynRFR24_nc.x6_1
atgggcagcagccatcaccatcatcatcatagcagcggtctggttccgcgtggtagccgtatgcgtcgtgatgaaattctggaagaatatcgtcgtggtcgtcgtaactttcagcatattaatctgcaagaaatcgaactgaccaatgcaagcctgaccggtgccgatctgagctatgcaaatctgcatcatgccaatctgagccgtgccaacctgcgttcagccgatctgcgtaatgcgaacctgagtcatgcgaatctgtcaggcgcaaacctggaagaagcaaatctggaagcagcgaacctgcgtggtgcggatctgcatgaagcaaacctgtcaggtgccgatttacaagaagccaacctgacacaggcaaatctgaaagacgcgaatctgagtgacgccaatctggaacaggcagacctggcaggcgctgatctgcagggtgcagttctggatggtgctaatctgcatggtgcgaatttgaataacgctaatctgagcgaagcaatgctgactcgtgctaatttagaacaggcggatctgagcggtgcacgtaccaccggtgcgcgtctggatgatgcggatttacgtggtgcaaccgttgatccggttctgtggcgtaccgcaagcctgcgtggcgctaaaatggaagaagaacagcgtcgcgaatatgaacgtgcccgtggtggtggcggttctcgcatgcgtagagatgaaatcttagaagagtaccgtcgcggacgtcgcaattttcaacatatcaacttacaagagatcgagctgacaaacgcatcactgacaggtgcagacctgtcttatgccaatttacatcatgcaaatttgtcgagagcgaatctgcgctcagcagatttacgcaacgcaaatctgtcccatgcaaacctgagcggagcaaatttagaggaagccaatttagaagccgcaaatcttcgcggtgccgacctgcacgaggctaacctgagtggcgcagatcttcaagaagcgaatttaacccaggccaatcttaaagatgccaacttatcagatgctaaccttgagcaggcagatttagcgggtgcagacttacagggtgccgtgttagatggtgcaaatttacacggtgcaaatcttaataacgcgaacttatctgaggccatgctgacacgcgcaaacttagagcaagcggatttatcaggtgcccgtacaacaggcgcacgtttagatgatgccgatcttcggggtgcgacagtggaccctgtgctgtggcgcacagccagcttacgcggtgccaagatggaagaggaacaacgccgtgagtacgaacgtgcacgcggtggcggtggcagtcggatgcgtcgggacgagattcttgaggaatacagacgcggtcgcagaaattttcagcacataaaccttcaagaaattgagttaaccaatgcctctttaaccggtgcggacttaagctatgccaaccttcatcacgcgaatttatcacgtgcgaaccttcgcagcgcagacctgcgcaacgctaatttaagccatgcgaacttaagcggtgcaaaccttgaggaagcgaaccttgaagctgcgaatttacgcggagctgatttacatgaggccaatttatctggggctgacttgcaagaggcaaacttaacgcaggctaacttaaaagacgcaaacctttcagacgccaaccttgaacaagccgatcttgctggtgcggaccttcaaggtgccgtgctggacggtgcgaacttgcatggggctaatcttaacaatgctaatctttccgaagccatgttaacccgtgctaacttggaacaagctgacttaagtggcgctcgcaccacaggtgcacgcctggacgacgcagaccttcgtggtgccacagtagatccagtgttatggcgcaccgcctcattacggggtgcaaaaatggaagaggaacaaagacgtgaatatgagcgtgctcgcggaggtggtggctctcgcatgcgacgcgacgaaattttagaggaatatcgcagaggtcgccgtaatttccaacacatcaatttgcaagaaatagagcttacgaatgcgtcattgactggggcagatctgagttacgctaacctgcaccacgcgaaccttagtcgggcaaacctgcgctctgcggatcttcggaacgccaacttgagccacgcaaatttaagtggtgcgaatctggaagaggccaacttagaggctgccaatcttagaggggcagacctgcatgaggcgaatctttcaggtgctgatctgcaagaggccaatctgacccaagccaacttgaaggatgcaaaccttagtgatgcaaatcttgagcaagctgatctggcaggcgcagatttacaaggtgcggtgcttgatggcgctaaccttcatggggcaaacttgaataatgccaacctgtcggaagctatgcttaccagagcgaacttggagcaggccgacctttctggtgcacgcacaacgggtgctagactggatgacgccgacttaagaggtgcgacggttgatcctgttttatggcggacagcaagtttaagaggcgcaaagatggaagaggaacagcgaagagaatatgaaagagcacgcggtggtggcggttctcgcatgcgtagagatgaaatcttagaagagtaccgtcgcggacgtcgcaattttcaacatatcaacttacaagagatcgagctgacaaacgcatcactgacaggtgcagacctgtcttatgccaatttacatcatgcaaatttgtcgagagcgaatctgcgctcagcagatttacgcaacgcaaatctgtcccatgcaaacctgagcggagcaaatttagaggaagccaatttagaagccgcaaatcttcgcggtgccgacctgcacgaggctaacctgagtggcgcagatcttcaagaagcgaatttaacccaggccaatcttaaagatgccaacttatcagatgctaaccttgagcaggcagatttagcgggtgcagacttacagggtgccgtgttagatggtgcaaatttacacggtgcaaatcttaataacgcgaacttatctgaggccatgctgacacgcgcaaacttagagcaagcggatttatcaggtgcccgtacaacaggcgcacgtttagatgatgccgatcttcggggtgcgacagtggaccctgtgctgtggcgcacagccagcttacgcggtgccaagatggaagaggaacaacgccgtgagtacgaacgtgcacgcggtggcggtggcagtcggatgcgtcgggacgagattcttgaggaatacagacgcggtcgcagaaattttcagcacataaaccttcaagaaattgagttaaccaatgcctctttaaccggtgcggacttaagctatgccaaccttcatcacgcgaatttatcacgtgcgaaccttcgcagcgcagacctgcgcaacgctaatttaagccatgcgaacttaagcggtgcaaaccttgaggaagcgaaccttgaagctgcgaatttacgcggagctgatttacatgaggccaatttatctggggctgacttgcaagaggcaaacttaacgcaggctaacttaaaagacgcaaacctttcagacgccaaccttgaacaagccgatcttgctggtgcggaccttcaaggtgccgtgctggacggtgcgaacttgcatggggctaatcttaacaatgctaatctttccgaagccatgttaacccgtgctaacttggaacaagctgacttaagtggcgctcgcaccacaggtgcacgcctggacgacgcagaccttcgtggtgccacagtagatccagtgttatggcgcaccgcctcattacggggtgcaaaaatggaagaggaacaaagacgtgaatatgagcgtgctcgcggaaaatcagatgatggttaa

SEQ ID NO: 172 - protein, 450 aa, Artificial Sequence
  SynRFR24_nc.x2_1
MGSSHHHHHHSSGLVPRGSRMRRDEILEEYRRGRRNFQHINLQEIELTNASLTGADLSYANLHHANLSRANLRSADLRNANLSHANLSGANLEEANLEAANLRGADLHEANLSGADLQEANLTQANLKDANLSDANLEQADLAGADLQGAVLDGANLHGANLNNANLSEAMLTRANLEQADLSGARTTGARLDDADLRGATVDPVLWRTASLRGAKMEEEQRREYERARGGGGSRMRRDEILEEYRRGRRNFQHINLQEIELTNASLTGADLSYANLHHANLSRANLRSADLRNANLSHANLSGANLEEANLEAANLRGADLHEANLSGADLQEANLTQANLKDANLSDANLEQADLAGADLQGAVLDGANLHGANLNNANLSEAMLTRANLEQADLSGARTTGARLDDADLRGATVDPVLWRTASLRGAKMEEEQRREYERARGKSDDG

SEQ ID NO: 173 - DNA, 1353 bp, Artificial Sequence
  SynRFR24_nc.x2_1
atgggcagcagccatcaccatcatcatcatagcagcggtctggttccgcgtggtagccgtatgcgtcgtgatgaaattctggaagaatatcgtcgtggtcgtcgtaactttcagcatattaatctgcaagaaatcgaactgaccaatgcaagcctgaccggtgccgatctgagctatgcaaatctgcatcatgccaatctgagccgtgccaacctgcgttcagccgatctgcgtaatgcgaacctgagtcatgcgaatctgtcaggcgcaaacctggaagaagcaaatctggaagcagcgaacctgcgtggtgcggatctgcatgaagcaaacctgtcaggtgccgatttacaagaagccaacctgacacaggcaaatctgaaagacgcgaatctgagtgacgccaatctggaacaggcagacctggcaggcgctgatctgcagggtgcagttctggatggtgctaatctgcatggtgcgaatttgaataacgctaatctgagcgaagcaatgctgactcgtgctaatttagaacaggcggatctgagcggtgcacgtaccaccggtgcgcgtctggatgatgcggatttacgtggtgcaaccgttgatccggttctgtggcgtaccgcaagcctgcgtggcgctaaaatggaagaagaacagcgtcgcgaatatgaacgtgcccgtggtggtggcggttctcgcatgcgtagagatgaaatcttagaagagtaccgtcgcggacgtcgcaattttcaacatatcaacttacaagagatcgagctgacaaacgcatcactgacaggtgcagacctgtcttatgccaatttacatcatgcaaatttgtcgagagcgaatctgcgctcagcagatttacgcaacgcaaatctgtcccatgcaaacctgagcggagcaaatttagaggaagccaatttagaagccgcaaatcttcgcggtgccgacctgcacgaggctaacctgagtggcgcagatcttcaagaagcgaatttaacccaggccaatcttaaagatgccaacttatcagatgctaaccttgagcaggcagatttagcgggtgcagacttacagggtgccgtgttagatggtgcaaatttacacggtgcaaatcttaataacgcgaacttatctgaggccatgctgacacgcgcaaacttagagcaagcggatttatcaggtgcccgtacaacaggcgcacgtttagatgatgccgatcttcggggtgcgacagtggaccctgtgctgtggcgcacagccagcttacgcggtgccaagatggaagaggaacaacgccgtgagtacgaacgtgcacgcggtaaatcagatgatggttaa